European Patent Specification EP 3 985 024 B1, published May 6, 2026. Title: ADMINISTRATION OF AN ANTI-ACTIVIN-A COMPOUND TO A SUBJECT. Applicant: AMGEN INC. SANTA MARIA BIOTHERAPEUTICS, INC. The sequence listing filed with the application follows.

SEQUENCE LISTING (312 sequences)

SEQ ID NO: 1 - DNA, 402 bp, Homo sapiens
  CDS (1)..(402)
atgacggcgccctgggtggccctcgccctcctctggggatcgctgtgcgccggctctgggcgtggggaggctgagacacgggagtgcatctactacaacgccaactgggagctggagcgcaccaaccagagcggcctggagcgctgcgaaggcgagcaggacaagcggctgcactgctacgcctcctggcgcaacagctctggcaccatcgagctcgtgaagaagggctgctggctagatgacttcaactgctacgataggcaggagtgtgtggccactgaggagaacccccaggtgtacttctgctgctgtgaaggcaacttctgcaacgagcgcttcactcatttgccagaggctgggggcccggaagtcacgtacgagccacccccgacagcccccacc

SEQ ID NO: 2 - protein, 134 aa, Homo sapiens
MTAPWVALALLWGSLCAGSGRGEAETRECIYYNANWELERTNQSGLERCEGEQDKRLHCYASWRNSSGTIELVKKGCWLDDFNCYDRQECVATEENPQVYFCCCEGNFCNERFTHLPEAGGPEVTYEPPPTAPT

SEQ ID NO: 3 - DNA, 387 bp, Homo sapiens
  CDS (1)..(387)
atggagtttgggctgagctgggttttcctcgttgctcttttaagaggtgtccagtgtgagacacggtggtgcatctactacaacgccaactgggagctggagcgcaccaaccagaccggcctggagcgctgcgaaggcgagcaggacaagcggctgcactgctacgcctcctggcgcaacagctctggcaccatcgagctcgtgaagaagggctgctggctagatgacttcaactgctacgataggcaggagtgtgtggccactgaggagaacccccaggtgtacttctgctgctgtgagggcaacttctgcaacgagcgcttcactcatttgccagaggctgggggcccggaagtcacgtacgagccacccccgacagcccccacc

SEQ ID NO: 4 - protein, 129 aa, Homo sapiens
MEFGLSWVFLVALLRGVQCETRWCIYYNANWELERTNQTGLERCEGEQDKRLHCYASWRNSSGTIELVKKGCWLDDFNCYDRQECVATEENPQVYFCCCEGNFCNERFTHLPEAGGPEVTYEPPPTAPT

SEQ ID NO: 5 - DNA, 330 bp, Homo sapiens
  CDS (1)..(330)
gagacacggtggtgcatctactacaacgccaactgggagctggagcgcaccaaccagaccggcctggagcgctgcgaaggcgagcaggacaagcggctgcactgctacgcctcctggcgcaacagctctggcaccatcgagctcgtgaagaagggctgctggctagatgacttcaactgctacgataggcaggagtgtgtggccactgaggagaacccccaggtgtacttctgctgctgtgagggcaacttctgcaacgagcgcttcactcatttgccagaggctgggggcccggaagtcacgtacgagccacccccgacagcccccacc

SEQ ID NO: 6 - protein, 110 aa, Homo sapiens
ETRWCIYYNANWELERTNQTGLERCEGEQDKRLHCYASWRNSSGTIELVKKGCWLDDFNCYDRQECVATEENPQVYFCCCEGNFCNERFTHLPEAGGPEVTYEPPPTAPT

SEQ ID NO: 7 - DNA, 1071 bp, Homo sapiens
  CDS (1)..(1071)
atggagtttgggctgagctgggttttcctcgttgctcttttaagaggtgtccagtgtgagacacggtggtgcatctactacaacgccaactgggagctggagcgcaccaaccagaccggcctggagcgctgcgaaggcgagcaggacaagcggctgcactgctacgcctcctggcgcaacagctctggcaccatcgagctcgtgaagaagggctgctggctagatgacttcaactgctacgataggcaggagtgtgtggccactgaggagaacccccaggtgtacttctgctgctgtgagggcaacttctgcaacgagcgcttcactcatttgccagaggctgggggcccggaagtcacgtacgagccacccccgacagcccccaccggagggggaggatctgtcgagtgcccaccgtgcccagcaccacctgtggcaggaccgtcagtcttcctcttccccccaaaacccaaggacaccctcatgatctcccggacccctgaggtcacgtgcgtggtggtggacgtgagccacgaagaccccgaggtccagttcaactggtacgtggacggcgtggaggtgcataatgccaagacaaagccacgggaggagcagttcaacagcacgttccgtgtggtcagcgtcctcaccgttgtgcaccaggactggctgaacggcaaggagtacaagtgcaaggtctccaacaaaggcctcccagcccccatcgagaaaaccatctccaaaaccaaagggcagccccgagaaccacaggtgtacaccctgcccccatcccgggaggagatgaccaagaaccaggtcagcctgacctgcctggtcaaaggcttctatcccagcgacatcgccgtggagtgggagagcaatgggcagccggagaacaactacaagaccacacctcccatgctggactccgacggctccttcttcctctacagcaagctcaccgtggacaagagcaggtggcagcaggggaacgtcttctcatgctccgtgatgcatgaggctctgcacaaccactacacgcagaagagcctctccctgtctccgggtaaa

SEQ ID NO: 8 - protein, 357 aa, Homo sapiens
MEFGLSWVFLVALLRGVQCETRWCIYYNANWELERTNQTGLERCEGEQDKRLHCYASWRNSSGTIELVKKGCWLDDFNCYDRQECVATEENPQVYFCCCEGNFCNERFTHLPEAGGPEVTYEPPPTAPTGGGGSVECPPCPAPPVAGPSVFLFPPKPKDTLMISRTPEVTCVVVDVSHEDPEVQFNWYVDGVEVHNAKTKPREEQFNSTFRVVSVLTVVHQDWLNGKEYKCKVSNKGLPAPIEKTISKTKGQPREPQVYTLPPSREEMTKNQVSLTCLVKGFYPSDIAVEWESNGQPENNYKTTPPMLDSDGSFFLYSKLTVDKSRWQQGNVFSCSVMHEALHNHYTQKSLSLSPGK

SEQ ID NO: 9 - DNA, 1014 bp, Homo sapiens
  CDS (1)..(1014)
gagacacggtggtgcatctactacaacgccaactgggagctggagcgcaccaaccagaccggcctggagcgctgcgaaggcgagcaggacaagcggctgcactgctacgcctcctggcgcaacagctctggcaccatcgagctcgtgaagaagggctgctggctagatgacttcaactgctacgataggcaggagtgtgtggccactgaggagaacccccaggtgtacttctgctgctgtgagggcaacttctgcaacgagcgcttcactcatttgccagaggctgggggcccggaagtcacgtacgagccacccccgacagcccccaccggagggggaggatctgtcgagtgcccaccgtgcccagcaccacctgtggcaggaccgtcagtcttcctcttccccccaaaacccaaggacaccctcatgatctcccggacccctgaggtcacgtgcgtggtggtggacgtgagccacgaagaccccgaggtccagttcaactggtacgtggacggcgtggaggtgcataatgccaagacaaagccacgggaggagcagttcaacagcacgttccgtgtggtcagcgtcctcaccgttgtgcaccaggactggctgaacggcaaggagtacaagtgcaaggtctccaacaaaggcctcccagcccccatcgagaaaaccatctccaaaaccaaagggcagccccgagaaccacaggtgtacaccctgcccccatcccgggaggagatgaccaagaaccaggtcagcctgacctgcctggtcaaaggcttctatcccagcgacatcgccgtggagtgggagagcaatgggcagccggagaacaactacaagaccacacctcccatgctggactccgacggctccttcttcctctacagcaagctcaccgtggacaagagcaggtggcagcaggggaacgtcttctcatgctccgtgatgcatgaggctctgcacaaccactacacgcagaagagcctctccctgtctccgggtaaa

SEQ ID NO: 10 - protein, 338 aa, Homo sapiens
ETRWCIYYNANWELERTNQTGLERCEGEQDKRLHCYASWRNSSGTIELVKKGCWLDDFNCYDRQECVATEENPQVYFCCCEGNFCNERFTHLPEAGGPEVTYEPPPTAPTGGGGSVECPPCPAPPVAGPSVFLFPPKPKDTLMISRTPEVTCVVVDVSHEDPEVQFNWYVDGVEVHNAKTKPREEQFNSTFRVVSVLTVVHQDWLNGKEYKCKVSNKGLPAPIEKTISKTKGQPREPQVYTLPPSREEMTKNQVSLTCLVKGFYPSDIAVEWESNGQPENNYKTTPPMLDSDGSFFLYSKLTVDKSRWQQGNVFSCSVMHEALHNHYTQKSLSLSPGK

SEQ ID NO: 11 - DNA, 387 bp, Homo sapiens
  CDS (1)..(387)
atggagtttgggctgagctgggttttcctcgttgctcttttaagaggtgtccagtgtgagacacggtactgcatctactacaacgccaactgggagctggagcgcaccaaccagaccggcctggagcgctgcgaaggcgagcaggacaagcggctgcactgctacgcctcctggcgcaacagctctggcaccatcgagctcgtgaagaagggctgctggctagatgacttcaactgctacgataggcaggagtgtgtggccactgaggagaacccccaggtgtacttctgctgctgtgagggcaacttctgcaacgagcgcttcactcatttgccagaggctgggggcccggaagtcacgtacgagccacccccgacagcccccacc

SEQ ID NO: 12 - protein, 129 aa, Homo sapiens
MEFGLSWVFLVALLRGVQCETRYCIYYNANWELERTNQTGLERCEGEQDKRLHCYASWRNSSGTIELVKKGCWLDDFNCYDRQECVATEENPQVYFCCCEGNFCNERFTHLPEAGGPEVTYEPPPTAPT

SEQ ID NO: 13 - DNA, 330 bp, Homo sapiens
  CDS (1)..(330)
gagacacggtactgcatctactacaacgccaactgggagctggagcgcaccaaccagaccggcctggagcgctgcgaaggcgagcaggacaagcggctgcactgctacgcctcctggcgcaacagctctggcaccatcgagctcgtgaagaagggctgctggctagatgacttcaactgctacgataggcaggagtgtgtggccactgaggagaacccccaggtgtacttctgctgctgtgagggcaacttctgcaacgagcgcttcactcatttgccagaggctgggggcccggaagtcacgtacgagccacccccgacagcccccacc

SEQ ID NO: 14 - protein, 110 aa, Homo sapiens
ETRYCIYYNANWELERTNQTGLERCEGEQDKRLHCYASWRNSSGTIELVKKGCWLDDFNCYDRQECVATEENPQVYFCCCEGNFCNERFTHLPEAGGPEVTYEPPPTAPT

SEQ ID NO: 15 - DNA, 1071 bp, Homo sapiens
  CDS (1)..(1071)
atggagtttgggctgagctgggttttcctcgttgctcttttaagaggtgtccagtgtgagacacggtactgcatctactacaacgccaactgggagctggagcgcaccaaccagaccggcctggagcgctgcgaaggcgagcaggacaagcggctgcactgctacgcctcctggcgcaacagctctggcaccatcgagctcgtgaagaagggctgctggctagatgacttcaactgctacgataggcaggagtgtgtggccactgaggagaacccccaggtgtacttctgctgctgtgagggcaacttctgcaacgagcgcttcactcatttgccagaggctgggggcccggaagtcacgtacgagccacccccgacagcccccaccggagggggaggatctgtcgagtgcccaccgtgcccagcaccacctgtggcaggaccgtcagtcttcctcttccccccaaaacccaaggacaccctcatgatctcccggacccctgaggtcacgtgcgtggtggtggacgtgagccacgaagaccccgaggtccagttcaactggtacgtggacggcgtggaggtgcataatgccaagacaaagccacgggaggagcagttcaacagcacgttccgtgtggtcagcgtcctcaccgttgtgcaccaggactggctgaacggcaaggagtacaagtgcaaggtctccaacaaaggcctcccagcccccatcgagaaaaccatctccaaaaccaaagggcagccccgagaaccacaggtgtacaccctgcccccatcccgggaggagatgaccaagaaccaggtcagcctgacctgcctggtcaaaggcttctatcccagcgacatcgccgtggagtgggagagcaatgggcagccggagaacaactacaagaccacacctcccatgctggactccgacggctccttcttcctctacagcaagctcaccgtggacaagagcaggtggcagcaggggaacgtcttctcatgctccgtgatgcatgaggctctgcacaaccactacacgcagaagagcctctccctgtctccgggtaaa

SEQ ID NO: 16 - protein, 357 aa, Homo sapiens
MEFGLSWVFLVALLRGVQCETRYCIYYNANWELERTNQTGLERCEGEQDKRLHCYASWRNSSGTIELVKKGCWLDDFNCYDRQECVATEENPQVYFCCCEGNFCNERFTHLPEAGGPEVTYEPPPTAPTGGGGSVECPPCPAPPVAGPSVFLFPPKPKDTLMISRTPEVTCVVVDVSHEDPEVQFNWYVDGVEVHNAKTKPREEQFNSTFRVVSVLTVVHQDWLNGKEYKCKVSNKGLPAPIEKTISKTKGQPREPQVYTLPPSREEMTKNQVSLTCLVKGFYPSDIAVEWESNGQPENNYKTTPPMLDSDGSFFLYSKLTVDKSRWQQGNVFSCSVMHEALHNHYTQKSLSLSPGK

SEQ ID NO: 17 - DNA, 1014 bp, Homo sapiens
  CDS (1)..(1014)
gagacacggtactgcatctactacaacgccaactgggagctggagcgcaccaaccagaccggcctggagcgctgcgaaggcgagcaggacaagcggctgcactgctacgcctcctggcgcaacagctctggcaccatcgagctcgtgaagaagggctgctggctagatgacttcaactgctacgataggcaggagtgtgtggccactgaggagaacccccaggtgtacttctgctgctgtgagggcaacttctgcaacgagcgcttcactcatttgccagaggctgggggcccggaagtcacgtacgagccacccccgacagcccccaccggagggggaggatctgtcgagtgcccaccgtgcccagcaccacctgtggcaggaccgtcagtcttcctcttccccccaaaacccaaggacaccctcatgatctcccggacccctgaggtcacgtgcgtggtggtggacgtgagccacgaagaccccgaggtccagttcaactggtacgtggacggcgtggaggtgcataatgccaagacaaagccacgggaggagcagttcaacagcacgttccgtgtggtcagcgtcctcaccgttgtgcaccaggactggctgaacggcaaggagtacaagtgcaaggtctccaacaaaggcctcccagcccccatcgagaaaaccatctccaaaaccaaagggcagccccgagaaccacaggtgtacaccctgcccccatcccgggaggagatgaccaagaaccaggtcagcctgacctgcctggtcaaaggcttctatcccagcgacatcgccgtggagtgggagagcaatgggcagccggagaacaactacaagaccacacctcccatgctggactccgacggctccttcttcctctacagcaagctcaccgtggacaagagcaggtggcagcaggggaacgtcttctcatgctccgtgatgcatgaggctctgcacaaccactacacgcagaagagcctctccctgtctccgggtaaa

SEQ ID NO: 18 - protein, 338 aa, Homo sapiens
ETRYCIYYNANWELERTNQTGLERCEGEQDKRLHCYASWRNSSGTIELVKKGCWLDDFNCYDRQECVATEENPQVYFCCCEGNFCNERFTHLPEAGGPEVTYEPPPTAPTGGGGSVECPPCPAPPVAGPSVFLFPPKPKDTLMISRTPEVTCVVVDVSHEDPEVQFNWYVDGVEVHNAKTKPREEQFNSTFRVVSVLTVVHQDWLNGKEYKCKVSNKGLPAPIEKTISKTKGQPREPQVYTLPPSREEMTKNQVSLTCLVKGFYPSDIAVEWESNGQPENNYKTTPPMLDSDGSFFLYSKLTVDKSRWQQGNVFSCSVMHEALHNHYTQKSLSLSPGK

SEQ ID NO: 19 - protein, 110 aa, Homo sapiens
ETRWCIYYNANWELERTNQSGLERCEGEQDKRLHCYASWRNSSGTIELVKKGCWLDDFNCYDRQECVATEENPQVYFCCCEGNFCNERFTHLPEAGGPEVTYEPPPTAPT

SEQ ID NO: 20 - DNA, 1014 bp, Homo sapiens
  CDS (1)..(1014)
gagacacggtggtgcatctactacaacgccaactgggagctggagcgcaccaaccagagcggcctggagcgctgcgaaggcgagcaggacaagcggctgcactgctacgcctcctggcgcaacagctctggcaccatcgagctcgtgaagaagggctgctggctagatgacttcaactgctacgataggcaggagtgtgtggccactgaggagaacccccaggtgtacttctgctgctgtgagggcaacttctgcaacgagcgcttcactcatttgccagaggctgggggcccggaagtcacgtacgagccacccccgacagcccccaccggaggaggaggatctgtcgagtgcccaccgtgcccagcaccacctgtggcaggaccgtcagtcttcctcttccccccaaaacccaaggacaccctcatgatctcccggacccctgaggtcacgtgcgtggtggtggacgtgagccacgaagaccccgaggtccagttcaactggtacgtggacggcgtggaggtgcataatgccaagacaaagccacgggaggagcagttcaacagcacgttccgtgtggtcagcgtcctcaccgttgtgcaccaggactggctgaacggcaaggagtacaagtgcaaggtctccaacaaaggcctcccagcccccatcgagaaaaccatctccaaaaccaaagggcagccccgagaaccacaggtgtacaccctgcccccatcccgggaggagatgaccaagaaccaggtcagcctgacctgcctggtcaaaggcttctatcccagcgacatcgccgtggagtgggagagcaatgggcagccggagaacaactacaagaccacacctcccatgctggactccgacggctccttcttcctctacagcaagctcaccgtggacaagagcaggtggcagcaggggaacgtcttctcatgctccgtgatgcatgaggctctgcacaaccactacacgcagaagagcctctccctgtctccgggtaaa

SEQ ID NO: 21 - protein, 338 aa, Homo sapiens
ETRWCIYYNANWELERTNQSGLERCEGEQDKRLHCYASWRNSSGTIELVKKGCWLDDFNCYDRQECVATEENPQVYFCCCEGNFCNERFTHLPEAGGPEVTYEPPPTAPTGGGGSVECPPCPAPPVAGPSVFLFPPKPKDTLMISRTPEVTCVVVDVSHEDPEVQFNWYVDGVEVHNAKTKPREEQFNSTFRVVSVLTVVHQDWLNGKEYKCKVSNKGLPAPIEKTISKTKGQPREPQVYTLPPSREEMTKNQVSLTCLVKGFYPSDIAVEWESNGQPENNYKTTPPMLDSDGSFFLYSKLTVDKSRWQQGNVFSCSVMHEALHNHYTQKSLSLSPGK

SEQ ID NO: 22 - protein, 216 aa, Homo sapiens
APPVAGPSVFLFPPKPKDTLMISRTPEVTCVVVDVSHEDPEVQFNWYVDGVEVHNAKTKPREEQFNSTFRVVSVLTVVHQDWLNGKEYKCKVSNKGLPAPIEKTISKTKGQPREPQVYTLPPSREEMTKNQVSLTCLVKGFYPSDIAVEWESNGQPENNYKTTPPMLDSDGSFFLYSKLTVDKSRWQQGNVFSCSVMHEALHNHYTQKSLSLSPGK

SEQ ID NO: 23 - protein, 217 aa, Homo sapiens
APELLGGPSVFLFPPKPKDILMISRTPEVTCVVVDVSHEDPEVKFNWYVGGVEVHNAKTKPREEQYNSTYRVVSVLTVLHQDWLNGKEYKCKVSNKALPAPIEKTISKAKGQPREPQVYTLPPSRDELTKNQVSLTCLVKGFYPSDIAVEWESNGQPENNYKTTPPVLDSDGSFFLYSKLTVDKSRWQQGNVFSCSVMHEALHNHYTQKSLSLSPGK

SEQ ID NO: 24 - protein, 217 aa, Homo sapiens
APEFLGGPSVFLFPPKPKDTLMISRTPEVTCVVVDVSQEDPEVQFNWYVDGVEVHNAKTKPREEQFNSTYRVVSVLTVLHQDWLNGKEYKCKVSNKGLPSSIEKTISKAKGQPREPQVYTLPPSQEEMTKNQVSLTCLVKGFYPSDIAVEWESNGQPENNYKTTPPVLDSDGSFFLYSRLTVDKSRWQEGNVFSCSVMHEALHNHYTQKSLSLSLGK

SEQ ID NO: 25 - protein, 5 aa, Artificial Sequence
  Description of Artificial Sequence: Synthetic linker peptide
GGGGS

SEQ ID NO: 26 - DNA, 36 bp, Artificial Sequence
  Description of Artificial Sequence: Synthetic hinge linker oligonucleotide
  CDS (1)..(36)
ggagggggaggatctgtcgagtgcccaccgtgccca

SEQ ID NO: 27 - protein, 12 aa, Artificial Sequence
  Description of Artificial Sequence: Synthetic hinge linker peptide
GGGGSVECPPCP

SEQ ID NO: 28 - protein, 12 aa, Homo sapiens
ERKCCVECPPCP

SEQ ID NO: 29 - protein, 15 aa, Homo sapiens
EPKSCDKTHTCPPCP

SEQ ID NO: 30 - protein, 12 aa, Homo sapiens
ESKTGPPCPSCP

SEQ ID NO: 31 - protein, 18 aa, Homo sapiens
MTAPWVALALLWGSLWPG

SEQ ID NO: 32 - protein, 18 aa, Homo sapiens
MTAPWVALALLWGSLCAG

SEQ ID NO: 33 - protein, 512 aa, Homo sapiens
MTAPWVALALLWGSLCAGSGRGEAETRECIYYNANWELERTNQSGLERCEGEQDKRLHCYASWRNSSGTIELVKKGCWLDDFNCYDRQECVATEENPQVYFCCCEGNFCNERFTHLPEAGGPEVTYEPPPTAPTLLTVLAYSLLPIGGLSLIVLLAFWMYRHRKPPYGHVDIHEDPGPPPPSPLVGLKPLQLLEIKARGRFGCVWKAQLMNDFVAVKIFPLQDKQSWQSEREIFSTPGMKHENLLQFIAAEKRGSNLEVELWLITAFHDKGSLTDYLKGNIITWNELCHVAETMSRGLSYLHEDVPWCRGEGHKPSIAHRDFKSKNVLLKSDLTAVLADFGLAVRFEPGKPPGDTHGQVGTRRYMAPEVLEGAINFQRDAFLRIDMYAMGLVLWELVSRCKAADGPVDEYMLPFEEEIGQHPSLEELQEVVVHKKMRPTIKDHWLKHPGLAQLCVTIEECWDHDAEARLSAGCVEERVSLIRRSVNGTTSDCLVSLVTSVTNVDLPPKESSI

SEQ ID NO: 34 - protein, 426 aa, Homo sapiens
MPLLWLRGFLLASCWIIVRSSPTPGSEGHSAAPDCPSCALAALPKDVPNSQPEMVEAVKKHILNMLHLKKRPDVTQPVPKAALLNAIRKLHVGKVGENGYVEIEDDIGRRAEMNELMEQTSEIITFAESGTARKTLHFEISKEGSDLSVVERAEVWLFLKVPKANRTRTKVTIRLFQQQKHPQGSLDTGEEAEEVGLKGERSELLLSEKVVDARKSTWHVFPVSSSIQRLLDQGKSSLDVRIACEQCQESGASLVLLGKKKKKEEEGEGKKKGGGEGGAGADEEKEQSHRPFLMLQARQSEDHPHRRRRRGLECDGKVNICCKKQFFVSFKDIGWNDWIIAPSGYHANYCEGECPSHIAGTSGSSLSFHSTVINHYRMRGHSPFANLKSCCVPTKLRPMSMLYYDDGQNIIKKDIQNMIVEECGCS

SEQ ID NO: 35 - protein, 375 aa, Homo sapiens
MQKLQLCVYIYLFMLIVAGPVDLNENSEQKENVEKEGLCNACTWRQNTKSSRIEAIKIQILSKLRLETAPNISKDVIRQLLPKAPPLRELIDQYDVQRDDSSDGSLEDDDYHATTETIITMPTESDFLMQVDGKPKCCFFKFSSKIQYNKVVKAQLWIYLRPVETPTTVFVQILRLIKPMKDGTRYTGIRSLKLDMNPGTGIWQSIDVKTVLQNWLKQPESNLGIEIKALDENGHDLAVTFPGPGEDGLNPFLEVKVTDTPKRSRRDFGLDCDEHSTESRCCRYPLTVDFEAFGWDWIIAPKRYKANYCSGECEFVFLQKYPHTHLVHQANPRGSAGPCCTPTKMSPINMLYFNGKEQIIYGKIPAMVVDRCGCS

SEQ ID NO: 36 - protein, 217 aa, Homo sapiens; identical to SEQ ID NO: 23

SEQ ID NO: 37 - DNA, 48 bp, Artificial Sequence
  Description of Artificial Sequence: Synthetic hinge linker oligonucleotide
  CDS (1)..(48)
ggagggggaggatctgagcgcaaatgttgtgtcgagtgcccaccgtgc

SEQ ID NO: 38 - protein, 16 aa, Artificial Sequence
  Description of Artificial Sequence: Synthetic hinge linker peptide
GGGGSERKCCVECPPC

SEQ ID NO: 39 - DNA, 42 bp, Artificial Sequence
  Description of Artificial Sequence: Synthetic hinge linker oligonucleotide
  CDS (1)..(42)
ggagggggaggatctggtggaggtggttcaggtccaccgtgc

SEQ ID NO: 40 - protein, 14 aa, Artificial Sequence
  Description of Artificial Sequence: Synthetic hinge linker eptide
GGGGSGGGGSGPPC

SEQ ID NO: 41 - DNA, 42 bp, Artificial Sequence
  Description of Artificial Sequence: Synthetic hinge linker oligonucleotide
  CDS (1)..(42)
ggagggggaggatctggtggaggtggttcaggtccaccggga

SEQ ID NO: 42 - protein, 14 aa, Artificial Sequence
  Description of Artificial Sequence: Synthetic hinge linker peptide
GGGGSGGGGSGPPG

SEQ ID NO: 43 - DNA, 54 bp, Artificial Sequence
  Description of Artificial Sequence: Synthetic hinge linker oligonucleotide
  CDS (1)..(54)
ggagggggaggatctgagcgcaaatgtccaccttgtgtcgagtgcccaccgtgc

SEQ ID NO: 44 - protein, 18 aa, Artificial Sequence
  Description of Artificial Sequence: Synthetic hinge linker peptide
GGGGSERKCPPCVECPPC

SEQ ID NO: 45 - protein, 14 aa, Artificial Sequence
  Description of Artificial Sequence: Synthetic hinge linker peptide
GPASGGPASGPPCP

SEQ ID NO: 46 - protein, 21 aa, Artificial Sequence
  Description of Artificial Sequence: Synthetic hinge linker peptide
GPASGGPASGCPPCVECPPCP

SEQ ID NO: 47 - protein, 217 aa, Homo sapiens
APELLGGPSVFLFPPKPKDTLMISRTPEVTCVVVDVSHEDPEVKFNWYVDGVEVHNAKTKPREEQYNSTYRVVSVLTVLHQDWLNGKEYKCKVSNKALPAPIEKTISKAKGQPREPQVYTLPPSREEMTKNQVSLTCLVKGFYPSDIAVEWESNGQPENNYKTTPPVLDSDGSFFLYSKLTVDKSRWQQGNVFSCSVMHEALHNHYTQKSLSLSPGK

SEQ ID NO: 48 - protein, 16 aa, Artificial Sequence
  Description of Artificial Sequence: Synthetic hinge linker peptide
GGGGSVDKTHTCPPCP

SEQ ID NO: 49 - protein, 16 aa, Artificial Sequence
  Description of Artificial Sequence: Synthetic hinge linker peptide
GGGGSVDKTHTGPPCP

SEQ ID NO: 50 - protein, 21 aa, Artificial Sequence
  Description of Artificial Sequence: Synthetic hinge linker peptide
GGGGSGGGGSVDKTHTGPPCP

SEQ ID NO: 51 - DNA, 48 bp, Homo sapiens
aggtctagtcagagcctcctgcatagtactggatacaactatttggat

SEQ ID NO: 52 - DNA, 21 bp, Homo sapiens
ttgggttcttttcgggcctcc

SEQ ID NO: 53 - DNA, 26 bp, Homo sapiens
atgcaagctctccaaactccgtgcag

SEQ ID NO: 54 - DNA, 30 bp, Homo sapiens
ggatacaccttcaccggctactatatccac

SEQ ID NO: 55 - DNA, 51 bp, Homo sapiens
tggatcaaccctaacagtggtggcacaaactatgcacagaagtttcagggc

SEQ ID NO: 56 - DNA, 36 bp, Homo sapiens
gattcggggtatagcagcagctggcactttgactac

SEQ ID NO: 57 - protein, 112 aa, Homo sapiens
DIVMTQSPLSLPVTPGEPASISCRSSQSLLHSTGYNYLDWYLQKPGQSPQLLIYLGSFRASGVPDRFSGSGSGTDFTLKISRVEAEDVGVYYCMQALQTPCSFGQGTKLEIK

SEQ ID NO: 58 - protein, 121 aa, Homo sapiens
QVQLVQSGAEVKKPGASVKVSCKASGYTFTGYYIHWVRQAPGQGLEWMGWINPNSGGTNYAQKFQGRVTMTRDTSISTAYMELSRLRSDDTAVYFCARDSGYSSSWHFDYWGQGTLVTVSS

SEQ ID NO: 59 - protein, 11 aa, Homo sapiens
SGDKLGDKYAC

SEQ ID NO: 60 - protein, 7 aa, Homo sapiens
QDSKRPS

SEQ ID NO: 61 - protein, 9 aa, Homo sapiens
QAWDSSTAV

SEQ ID NO: 62 - protein, 10 aa, Homo sapiens
GYTFTSYGLS

SEQ ID NO: 63 - protein, 17 aa, Homo sapiens
WIIPYNGNTNSAQKLQG

SEQ ID NO: 64 - protein, 13 aa, Homo sapiens
DRDYGVNYDAFDI

SEQ ID NO: 65 - DNA, 339 bp, Homo sapiens
gacatcgtgatgacccagtctccagactccctggctgtgtctctgggcgagagggccaccatcacctgcaagtccagccagagtattttatacagttccaacaataagaagtatctagtttggtaccagcagaaaccaggacagcctcctaagctgatcatttactggacatctatgcgggaatccggggtccctgaccgattcagtggcagcgggtctgggacagatttcactctcaccatcaacagcctgcaggctgaagatgtggcagtttattactgtcagcaatattatagtactccgtggacgttcggccaagggaccaaggtggaaatcaaa

SEQ ID NO: 66 - DNA, 488 bp, Homo sapiens
caggtgcagctgcaggagtcgggcccaggactggtgaagccttcggagaccctgtccctcacctgcactgtctctggtggctccatcaatagtttctactggagctggatccggcagcccccagggaagggactggagtggattgggtatatctattacagtgggagcaccaactacaatccctccctcaagagtcgagtcaccatatcagtagacacgtccaagacccagttctccctgaagctgagctctgtgaccgctgcggacacggccgtgtattactgtgcgagagacagtatagcagccccctttgactactggggccagggaaccctggtcaccgtctcctcagcttccaccaagggcccatccgtcttccccctggcgccctgctccaggagcacctccgagagcacagccgccctgggctgcctggtcaaggactacttccccgaaccggtgacggtgtcgtggaactcatgcgccct

SEQ ID NO: 67 - DNA, 51 bp, Homo sapiens
aagtccagccagagtattttatacagttccaacaataagaagtatctagtt

SEQ ID NO: 68 - DNA, 21 bp, Homo sapiens
tggacatctatgcgggaatcc

SEQ ID NO: 69 - DNA, 27 bp, Homo sapiens
cagcaatattatagtactccgtggacg

SEQ ID NO: 70 - DNA, 30 bp, Homo sapiens
ggtggctccatcaatagtttctactggagc

SEQ ID NO: 71 - DNA, 48 bp, Homo sapiens
tatatctattacagtgggagcaccaactacaatccctccctcaagagt

SEQ ID NO: 72 - DNA, 27 bp, Homo sapiens
gacagtatagcagccccctttgactac

SEQ ID NO: 73 - protein, 113 aa, Homo sapiens
DIVMTQSPDSLAVSLGERATITCKSSQSILYSSNNKKYLVWYQQKPGQPPKLIIYWTSMRESGVPDRFSGSGSGTDFTLTINSLQAEDVAVYYCQQYYSTPWTFGQGTKVEIK

SEQ ID NO: 74 - protein, 117 aa, Homo sapiens
QVQLQESGPGLVKPSETLSLTCTVSGGSINSFYWSWIRQPPGKGLEWIGYIYYSGSTNYNPSLKSRVTISVDTSKTQFSLKLSSVTAADTAVYYCARDSIAAPFDYWGQGTLVTVSS

SEQ ID NO: 75 - protein, 17 aa, Homo sapiens
KSSQSILYSSNNKKYLV

SEQ ID NO: 76 - protein, 7 aa, Homo sapiens
WTSMRES

SEQ ID NO: 77 - protein, 9 aa, Homo sapiens
QQYYSTPWT

SEQ ID NO: 78 - protein, 10 aa, Homo sapiens
GGSINSFYWS

SEQ ID NO: 79 - protein, 16 aa, Homo sapiens
YIYYSGSTNYNPSLKS

SEQ ID NO: 80 - protein, 9 aa, Homo sapiens
DSIAAPFDY

SEQ ID NO: 81 - DNA, 321 bp, Homo sapiens
gacatccagatgacccagtctccatcctccctgtctgcatctgtaggagacagagtcaccatcacttgccgggcaagtcagagcattagcaactatttaaattggtatcagcagagaccagggaaagcccctaagctcctgatctatgctacatccagtttgcaaagtggggtcccatcaaggttcagtggcagtggatctgggacagatttcactctcaccatcagcagtctgcaacctgaagattttgtaagttactactgtcaacagagttacagtatttcgcccactttcggcggcgggaccaaggtggagaacaaa

SEQ ID NO: 82 - DNA, 357 bp, Homo sapiens
caggtgcagctacagcagtggggcgcaggactgttgaagccttcggagaccctgtccctcacctgcgctgtctatggtgggtccttcagtgcttactactggagctggatccgccagcccccagggaagggactggagtggattggggaaatcaatcatagtggaggcaccaactacaacccgtccctcaagagtcgagtcaccatatcagtagacacgtccaagaaccagttctccctgaagctgagctctgtgaccgccgcggacacggctgtgtattactgtgcgagagtacagtggctcgaactggcctactttgactactggggccagggaaccctggtcaccgtctcctca

SEQ ID NO: 83 - DNA, 33 bp, Homo sapiens
cgggcaagtcagagcattagcaactatttaaat

SEQ ID NO: 84 - protein, 106 aa, Homo sapiens
GQPKAAPSVTLFPPSSEELQANKATLVCLISDFYPGAVTVAWKADSSPVKAGVETTTPSKQSNNKYAASSYLSLTPEQWKSHRSYSCQVTHEGSTVEKTVAPTECS

SEQ ID NO: 85 - DNA, 27 bp, Homo sapiens
caacagagttacagtatttcgcccact

SEQ ID NO: 86 - DNA, 30 bp, Homo sapiens
ggtgggtccttcagtgcttactactggagc

SEQ ID NO: 87 - DNA, 48 bp, Homo sapiens
gaaatcaatcatagtggaggcaccaactacaacccgtccctcaagagt

SEQ ID NO: 88 - DNA, 33 bp, Homo sapiens
gtacagtggctcgaactggcctactttgactac

SEQ ID NO: 89 - protein, 107 aa, Homo sapiens
DIQMTQSPSSLSASVGDRVTITCRASQSISNYLNWYQQRPGKAPKLLIYATSSLQSGVPSRFSGSGSGTDFTLTISSLQPEDFVSYYCQQSYSISPTFGGGTKVENK

SEQ ID NO: 90 - protein, 119 aa, Homo sapiens
QVQLQQWGAGLLKPSETLSLTCAVYGGSFSAYYWSWIRQPPGKGLEWIGEINHSGGTNYNPSLKSRVTISVDTSKNQFSLKLSSVTAADTAVYYCARVQWLELAYFDYWGQGTLVTVSS

SEQ ID NO: 91 - protein, 11 aa, Homo sapiens
RASQSISNYLN

SEQ ID NO: 92 - protein, 7 aa, Homo sapiens
ATSSLQS

SEQ ID NO: 93 - protein, 9 aa, Homo sapiens
QQSYSISPT

SEQ ID NO: 94 - protein, 10 aa, Homo sapiens
GGSFSAYYWS

SEQ ID NO: 95 - protein, 16 aa, Homo sapiens
EINHSGGTNYNPSLKS

SEQ ID NO: 96 - protein, 11 aa, Homo sapiens
VQWLELAYFDY

SEQ ID NO: 97 - DNA, 321 bp, Homo sapiens
gacatccagatgacccagtctccatcctccctgtctgcatctgtaggagacagagtcaccatcacttgccgggcaggtcagggcattagaaatgatttagtctggtatcagcagaaaccagggaaagcccctaagcgcctgatctatgctgcatccagtttgcaaagtggggtcccatcaaggttcagcggcagtggatctgggacagaattcactctcacaatcagcagcctgcagcctgaagattttgcaacttattactgtctacaacataatacttacccattcactttcggccctgggaccaaagtggatatcaaa

SEQ ID NO: 98 - DNA, 363 bp, Homo sapiens
caggtgcagctggtggactctgggggaggcgtggtccagcctgggaggtccctgagactctcctgtgcagcgtctggattcaccttcattagctatggcatgcactgggtccgccaggctccaggcaaggggctggagtgggtggcagttatctggtatgatggaagtactgaatactatgcagactccgtgaagggccgattcaccatctccagagacaattccaagaacacgctgtatctgcaaatgaacagcctgagagccgaggacacggctgtgtattactgtgcgagagagaggcagtggctctaccactacggtatggacgtctggggccaagggaccacggtcaccgtctcctca

SEQ ID NO: 99 - DNA, 33 bp, Homo sapiens
cgggcaggtcagggcattagaaatgatttagtc

SEQ ID NO: 100 - protein, 107 aa, Homo sapiens [sequence omitted]

SEQ ID NO: 101 - DNA, 27 bp, Homo sapiens
ctacaacataatacttacccattcact

SEQ ID NO: 102 - DNA, 30 bp, Homo sapiens
ggattcaccttcattagctatggcatgcac

SEQ ID NO: 103 - DNA, 51 bp, Homo sapiens
gttatctggtatgatggaagtactgaatactatgcagactccgtgaagggc

SEQ ID NO: 104 - DNA, 36 bp, Homo sapiens
gagaggcagtggctctaccactacggtatggacgtc

SEQ ID NO: 105 - protein, 107 aa, Homo sapiens
DIQMTQSPSSLSASVGDRVTITCRAGQGIRNDLVWYQQKPGKAPKRLIYAASSLQSGVPSRFSGSGSGTEFTLTISSLQPEDFATYYCLQHNTYPFTFGPGTKVDIK

SEQ ID NO: 106 - protein, 121 aa, Homo sapiens
QVQLVDSGGGVVQPGRSLRLSCAASGFTFISYGMHWVRQAPGKGLEWVAVIWYDGSTEYYADSVKGRFTISRDNSKNTLYLQMNSLRAEDTAVYYCARERQWLYHYGMDVWGQGTTVTVSS

SEQ ID NO: 107 - protein, 11 aa, Homo sapiens
RAGQGIRNDLV

SEQ ID NO: 108 - protein, 107 aa, Homo sapiens [sequence omitted]

SEQ ID NO: 109 - protein, 9 aa, Homo sapiens
LQHNTYPFT

SEQ ID NO: 110 - protein, 10 aa, Homo sapiens
GFTFISYGMH

SEQ ID NO: 111 - protein, 17 aa, Homo sapiens
VIWYDGSTEYYADSVKG

SEQ ID NO: 112 - protein, 12 aa, Homo sapiens
ERQWLYHYGMDV

SEQ ID NO: 113 - DNA, 339 bp, Homo sapiens
gacatcgtgatgacccagtctccagactccctggctgtgtctctgggcgagagggccaccatcacctgcaagtccagccagagtattttatacagctccaacaataagaagtatctagtttggtaccagcagaaaccaggacagcctcctaagttgatcatttactggacatctatgcgggaatccggggtccctgaccgattcagtggcagcgggtctgggacagatttcactctcaccatcagcagcctgcaggctgaagatgtggcagtttattactgtcagcaatattatagtactccgtggacgttcggccaagggaccaaggtggaaatcaaa

SEQ ID NO: 114 - DNA, 351 bp, Homo sapiens
caggtgcagctgcaggagtcgggcccaggactggtgaagccctcggagaccctgtccctcacctgcactgtctctggtggctccatcaatagtttctactggagctggatccggcagcccccagggaagggactggagtggattgggtatatctattacagtgggagcaccaactacaatccctccctcaagaggcgagtcaccatatcagtagacacgtccaagacccagttctccctgaagctgagctctgtgaccgctgcggacacggccgtgtattactgtgcgagagacagtatagcagccccctttgactactggggccagggaaccctggtcaccgtctcctca

SEQ ID NO: 115 - protein, 17 aa, Homo sapiens
  MOD_RES (1)..(1): Arg or Lys
  MOD_RES (6)..(6): Leu or Ile
  MOD_RES (8)..(8): His or Tyr
  MOD_RES (10)..(10): Thr or Ser
  MOD_RES (11)..(11): Gly or Asn
  MOD_RES (12)..(12): Tyr or Asn
  MOD_RES (13)..(13): Asn or Lys
  MOD_RES (14)..(14): May or may not be present
  MOD_RES (17)..(17): Asp or Val
XSSQSXLXSXXXXKYLX

SEQ ID NO: 116 - protein, 11 aa, Homo sapiens
  MOD_RES (3)..(3): Ser or Gly
  MOD_RES (5)..(5): Ser or Gly
  MOD_RES (7)..(7): Ser or Arg
  MOD_RES (9)..(9): Tyr, Asp or Asn
  MOD_RES (11)..(11): Asp, Val or Gly
RAXQXIXNXLX

SEQ ID NO: 117 - DNA, 27 bp, Homo sapiens
cagcaatattatagtactccgtggacg

SEQ ID NO: 118 - DNA, 30 bp, Homo sapiens; identical to SEQ ID NO: 70

SEQ ID NO: 119 - DNA, 48 bp, Homo sapiens
tatatctattacagtgggagcaccaactacaatccctccctcaagagg

SEQ ID NO: 120 - DNA, 27 bp, Homo sapiens
gacagtatagcagccccctttgactac

SEQ ID NO: 121 - protein, 113 aa, Homo sapiens
DIVMTQSPDSLAVSLGERATITCKSSQSILYSSNNKKYLVWYQQKPGQPPKLIIYWTSMRESGVPDRFSGSGSGTDFTLTISSLQAEDVAVYYCQQYYSTPWTFGQGTKVEIK

SEQ ID NO: 122 - protein, 117 aa, Homo sapiens
QVQLQESGPGLVKPSETLSLTCTVSGGSINSFYWSWIRQPPGKGLEWIGYIYYSGSTNYNPSLKRRVTISVDTSKTQFSLKLSSVTAADTAVYYCARDSIAAPFDYWGQGTLVTVSS

SEQ ID NO: 123 - protein, 11 aa, Homo sapiens
  MOD_RES (3)..(3): Glu or Asp
  MOD_RES (5)..(5): Trp or Leu
  MOD_RES (7)..(7): Glu or Asp
  MOD_RES (9)..(9): Tyr or Phe
  MOD_RES (10)..(10): Ala or Val
  MOD_RES (11)..(11): Cys or Phe
SGXKXGXKXXX

SEQ ID NO: 124 - protein, 7 aa, Homo sapiens
  MOD_RES (1)..(1): Ala, Trp or Leu
  MOD_RES (2)..(2): Thr, Ala or Gly
  MOD_RES (4)..(4): Ser, Met or Phe
  MOD_RES (5)..(5): Leu or Arg
  MOD_RES (6)..(6): Gln, Glu or Ala
XXSXXXS

SEQ ID NO: 125 - protein, 9 aa, Homo sapiens
QQYYSTPWT

SEQ ID NO: 126 - protein, 10 aa, Homo sapiens
GGSINSFYWS

SEQ ID NO: 127 - protein, 16 aa, Homo sapiens
YIYYSGSTNYNPSLKR

SEQ ID NO: 128 - protein, 7 aa, Homo sapiens
  MOD_RES (1)..(1): Gln, Leu or His
  MOD_RES (3)..(3): Thr, Asn or Ser
XDXKRPS

SEQ ID NO: 129 - DNA, 321 bp, Homo sapiens
gacatccagatgacccagtctccatcctccctgtctgcatctgtaggagacagagtcaccatcacttgccgggcaagtcagggcattagaaataatttaggctggtatcagcagaaaccagggaaagcccctaagcgcctgatttatgctgcatccagtttgcaaagtggggtcccatcaaggttcagcggcagtggatctgggacagaattcactctcacaatcagcagcctgcagcctgaagattttacaacttattactgtctacagcataatagttacccgtggacgttcggccaagggaccaaggtggaaatcaaa

SEQ ID NO: 130 - DNA, 372 bp, Homo sapiens
caggtgcagctggtggagtctgggggaggcgtggtccagcctgggaggtccctgagactctcctgtgcagcgtctggattcaccttcagtagttacggcatgcactgggtccgccaggctccaggcaaggggctggagtgggtggcagttatatggtatgatggaagtaataaataccatgcagactccgtgaagggccgattcaccatctccagagacaattccaagaacacgctgtatctgcaagtgaacagcctgagagccgaggacacggctgtgtattactgtgtgagaagtcggaactggaactacgacaactactactacggtctggacgtctggggccaagggaccacggtcaccgtctcctca

SEQ ID NO: 131 - protein, 9 aa, Homo sapiens
  MOD_RES (5)..(5): Thr or Ser
  MOD_RES (7)..(7): Pro or Thr
  MOD_RES (8)..(8): Phe or Trp
LQHNXYXXT

SEQ ID NO: 132 - protein, 9 aa, Homo sapiens
  MOD_RES (1)..(1): Met, Gln or Arg
  MOD_RES (3)..(3): Ala, Tyr, Gln or Ser
  MOD_RES (4)..(4): Leu, Tyr or Asn
  MOD_RES (5)..(5): Gln, Ser or Thr
  MOD_RES (6)..(6): Thr, Tyr or Ile
  MOD_RES (7)..(7): Pro or Ser
  MOD_RES (8)..(8): Cys, Trp, Leu or Pro
  MOD_RES (9)..(9): Ser or Thr
XQXXXXXXX

SEQ ID NO: 133 - DNA, 27 bp, Homo sapiens
ctacagcataatagttacccgtggacg

SEQ ID NO: 134 - protein, 11 aa, Homo sapiens
  MOD_RES (4)..(4): Ile or Phe
  MOD_RES (5)..(5): Asn or Ser
  MOD_RES (6)..(6): Ser or Ala
  MOD_RES (7)..(7): Gly or absent
  MOD_RES (8)..(8): Gly or absent
  MOD_RES (9)..(9): Phe or Tyr
GGSXXXXXXYW

SEQ ID NO: 135 - DNA, 51 bp, Homo sapiens
gttatatggtatgatggaagtaataaataccatgcagactccgtgaagggc

SEQ ID NO: 136 - DNA, 45 bp, Homo sapiens
agtcggaactggaactacgacaactactactacggtctggacgtc

SEQ ID NO: 137 - protein, 107 aa, Homo sapiens
DIQMTQSPSSLSASVGDRVTITCRASQGIRNNLGWYQQKPGKAPKRLIYAASSLQSGVPSRFSGSGSGTEFTLTISSLQPEDFTTYYCLQHNSYPWTFGQGTKVEIK

SEQ ID NO: 138 - protein, 124 aa, Homo sapiens
QVQLVESGGGVVQPGRSLRLSCAASGFTFSSYGMHWVRQAPGKGLEWVAVIWYDGSNKYHADSVKGRFTISRDNSKNTLYLQVNSLRAEDTAVYYCVRSRNWNYDNYYYGLDVWGQGTTVTVSS

SEQ ID NO: 139 - protein, 10 aa, Homo sapiens
  MOD_RES (2)..(2): Tyr or Phe
  MOD_RES (3)..(3): Tyr or Ser
  MOD_RES (5)..(5): Thr, Ser or Ile
  MOD_RES (6)..(6): Gly or Ser
  MOD_RES (8)..(8): Tyr, Gly or Trp
  MOD_RES (9)..(9): Ile or Met
  MOD_RES (10)..(10): His or Gly
GXXFXXYXXX

SEQ ID NO: 140 - protein, 10 aa, Homo sapiens
  MOD_RES (2)..(2): Tyr or Phe
  MOD_RES (5)..(5): Thr or Ser
  MOD_RES (6)..(6): Ser or Ala
  MOD_RES (8)..(8): Gly or Trp
  MOD_RES (9)..(9): Leu, Met or Ile
  MOD_RES (10)..(10): Ser or His
GXTFXXYXXX

SEQ ID NO: 141 - protein, 9 aa, Homo sapiens
LQHNSYPWT

SEQ ID NO: 142 - protein, 16 aa, Homo sapiens
  MOD_RES (1)..(1): Tyr or Glu
  MOD_RES (3)..(3): Ser, Tyr or Asn
  MOD_RES (4)..(4): Tyr or His
  MOD_RES (7)..(7): Ser or Gly
  MOD_RES (9)..(9): Tyr or Asn
  MOD_RES (16)..(16): Ser or Arg
XIXXSGXTXYNPSLKX

SEQ ID NO: 143 - protein, 17 aa, Homo sapiens
VIWYDGSNKYHADSVKG

SEQ ID NO: 144 - protein, 15 aa, Homo sapiens
SRNWNYDNYYYGLDV

SEQ ID NO: 145 - DNA, 315 bp, Homo sapiens
tcctatgagctgactcagccaccctcagtgtccgtgtccccaggacagacagccagcatcacctgctctggagaaaaatggggagagaaatatgcttgttggtatcagcagaagccaggccagtcccctgtgctggtcatctatcaagataccaagcggccctccgggatccctgagcgattctctggctccatttctgggaacacagccactctgaccatcagcgggacccaggctatggatgaggctgactattattgtcaggcgtgggacaggagcactgtattcggcggagggaccaagctgaccgtccta

SEQ ID NO: 146 - DNA, 348 bp, Homo sapiens
gaggtgcagctggtgcagtctggagcagaggtgaaaaagcccggggagtctctgaagatctcctgtcagggttctggatacagctttaccagctactggatcggctgggtgcgccagatgcccgggaaaggcctggagtggatggggatcatctatcctggtgactctgataccagatacagcccgtccttccaaggccaggtcaccatctcagccgacaagtccatcagcaccgcctacctgcagtggagcagcctgaaggcctcggacaccgccatgtattactgtgcgagacaaggactggggtttgactactggggccagggaaccctggtcaccgtctcctca

SEQ ID NO: 147 - DNA, 33 bp, Homo sapiens
tctggagaaaaatggggagagaaatatgcttgt

SEQ ID NO: 148 - DNA, 21 bp, Homo sapiens
caagataccaagcggccctcc

SEQ ID NO: 149 - DNA, 24 bp, Homo sapiens
caggcgtgggacaggagcactgta

SEQ ID NO: 150 - DNA, 30 bp, Homo sapiens
ggatacagctttaccagctactggatcggc

SEQ ID NO: 151 - DNA, 51 bp, Homo sapiens
atcatctatcctggtgactctgataccagatacagcccgtccttccaaggc

SEQ ID NO: 152 - DNA, 21 bp, Homo sapiens
caaggactggggtttgactac

SEQ ID NO: 153 - protein, 105 aa, Homo sapiens
SYELTQPPSVSVSPGQTASITCSGEKWGEKYACWYQQKPGQSPVLVIYQDTKRPSGIPERFSGSISGNTATLTISGTQAMDEADYYCQAWDRSTVFGGGTKLTVL

SEQ ID NO: 154 - protein, 116 aa, Homo sapiens
EVQLVQSGAEVKKPGESLKISCQGSGYSFTSYWIGWVRQMPGKGLEWMGIIYPGDSDTRYSPSFQGQVTISADKSISTAYLQWSSLKASDTAMYYCARQGLGFDYWGQGTLVTVSS

SEQ ID NO: 155 - protein, 11 aa, Homo sapiens
SGEKWGEKYAC

SEQ ID NO: 156 - protein, 7 aa, Homo sapiens
QDTKRPS

SEQ ID NO: 157 - protein, 8 aa, Homo sapiens
QAWDRSTV

SEQ ID NO: 158 - protein, 10 aa, Homo sapiens
GYSFTSYWIG

SEQ ID NO: 159 - protein, 17 aa, Homo sapiens
IIYPGDSDTRYSPSFQG

SEQ ID NO: 160 - protein, 7 aa, Homo sapiens
QGLGFDY

SEQ ID NO: 161 - DNA, 318 bp, Homo sapiens
tcctatgagctgactcagccaccctcagtgtccgtgtccccaggacagacagccagcatcacctgctctggagataaattgggggataaatttgctttctggtatcagctgaagccaggccagtcccctgtgctggtcatctatcaagataacaagcggccctcagggatccctgagcgattctctggctccaactctgggaacacagccactctgaccatcagcgggacccaggctatggatgcggctgacttttactgtcaggcgtgggacagcagcactgtggtattcggcggagggaccaagctgaccgtccta

SEQ ID NO: 162 - DNA, 363 bp, Homo sapiens
caggtgcagctgcaggagtcgggcccaggactggtgaagccttcacagaccctgtccctcacctgcactgtctctggtggctccatcagcagtggtggttactactggagctggatccgccagcacccagggaagggcctggagtggattgggtacatctcttacagtgggagcacctactacaacccgtccctcaagagtcgagttaccatatcagttgacacgtctaagaaccagttctccctgaagctgaactctgtgactgccgcggacacggccgtgtattactgtgcgcgcgcttacggtgactatcgcggctggttcgacccctggggccagggaaccctggtcaccgtctcctca

SEQ ID NO: 163 - DNA, 33 bp, Homo sapiens
tctggagataaattgggggataaatttgctttc

SEQ ID NO: 164 - DNA, 21 bp, Homo sapiens
caagataacaagcggccctca

SEQ ID NO: 165 - DNA, 27 bp, Homo sapiens
caggcgtgggacagcagcactgtggta

SEQ ID NO: 166 - DNA, 36 bp, Homo sapiens
ggtggctccatcagcagtggtggttactactggagc

SEQ ID NO: 167 - DNA, 48 bp, Homo sapiens
tacatctcttacagtgggagcacctactacaacccgtccctcaagagt

SEQ ID NO: 168 - DNA, 33 bp, Homo sapiens
gcttacggtgactatcgcggctggttcgacccc

SEQ ID NO: 169 - protein, 106 aa, Homo sapiens
SYELTQPPSVSVSPGQTASITCSGDKLGDKFAFWYQLKPGQSPVLVIYQDNKRPSGIPERFSGSNSGNTATLTISGTQAMDAADFYCQAWDSSTVVFGGGTKLTVL

SEQ ID NO: 170 - protein, 121 aa, Homo sapiens
QVQLQESGPGLVKPSQTLSLTCTVSGGSISSGGYYWSWIRQHPGKGLEWIGYISYSGSTYYNPSLKSRVTISVDTSKNQFSLKLNSVTAADTAVYYCARAYGDYRGWFDPWGQGTLVTVSS

SEQ ID NO: 171 - protein, 11 aa, Homo sapiens
SGDKLGDKFAF

SEQ ID NO: 172 - protein, 7 aa, Homo sapiens
QDNKRPS

SEQ ID NO: 173 - protein, 9 aa, Homo sapiens
QAWDSSTVV

SEQ ID NO: 174 - protein, 12 aa, Homo sapiens
GGSISSGGYYWS

SEQ ID NO: 175 - protein, 16 aa, Homo sapiens
YISYSGSTYYNPSLKS

SEQ ID NO: 176 - protein, 11 aa, Homo sapiens
AYGDYRGWFDP

SEQ ID NO: 177 - DNA, 321 bp, Homo sapiens
gacatccagatgacccagtctccatcctccctgtctgcatctgtaggagacagagtcaccatcacttgccgggcaagtcagggcattagaaatgatttaggctggtatcagcagaaaccagggaaagcccctaagcgcctgatctatgctgcatccagtttgcaaagtggggtcccatcaaggttcagcggcagtggatctgggacagaattcactctcacaatcagcagcctgcagcctgaagattgtgcaacttattattgtctacagcataatagttatacgtggacgttcggccaagggaccaaggtggaaatcaaa

SEQ ID NO: 178 - DNA, 372 bp, Homo sapiens
caggtgcagctggtggagtctgggggaggcgtggtccagcctgggaggtccctgagactctcctgtgtagcgtctggattcaccttcagtgcctatggcatgcactgggtccgccaggctccaggcaaggggctggagtgggtggcagttatatggtatgatggaagtaataaatactatgcagactccgtgaagggccgattcatcatctccagagacaattccaagaacacgctgtatctgcaaatgaacagcctgagagccgaggacacggctgtgtattactgtgcgagaagtcggaactggaactacgactcctaccaatacggtttggacgtctggggccaagggaccacggtcaccgtctcctca

SEQ ID NO: 179 - protein, 17 aa, Homo sapiens
  MOD_RES (1)..(1): Asn or Val
  MOD_RES (3)..(3): Trp or Lys
  MOD_RES (4)..(4): Tyr or Gln
  MOD_RES (8)..(8): Asn, Glu or Ser
  MOD_RES (9)..(9): Lys or Glu
  MOD_RES (11)..(11): His or Tyr
  MOD_RES (12)..(12): Ala or Val
XIXXDGSXXYXXDSVKG

SEQ ID NO: 180 - protein, 17 aa, Homo sapiens
  MOD_RES (1)..(1): Trp or Ile
  MOD_RES (3)..(3): Asn, Ile, Ser or Tyr
  MOD_RES (4)..(4): Pro or Ala
  MOD_RES (5)..(5): Asn, Tyr or Gly
  MOD_RES (6)..(6): Ser, Asn or Asp
  MOD_RES (7)..(7): Gly or Ser
  MOD_RES (8)..(8): Gly, Asn or Asp
  MOD_RES (10)..(10): Asn or Arg
  MOD_RES (11)..(11): Tyr or Ser
  MOD_RES (12)..(12): Ala or Ser
  MOD_RES (13)..(13): Gln or Pro
  MOD_RES (14)..(14): Lys or Ser
  MOD_RES (15)..(15): Phe or Leu
XIXXXXXXTXXXXXXQG

SEQ ID NO: 181 - DNA, 27 bp, Homo sapiens
ctacagcataatagttatacgtggacg

SEQ ID NO: 182 - DNA, 30 bp, Homo sapiens
ggattcaccttcagtgcctatggcatgcac

SEQ ID NO: 183 - DNA, 51 bp, Homo sapiens
gttatatggtatgatggaagtaataaatactatgcagactccgtgaagggc

SEQ ID NO: 184 - DNA, 45 bp, Homo sapiens
agtcggaactggaactacgactcctaccaatacggtttggacgtc

SEQ ID NO: 185 - protein, 107 aa, Homo sapiens
DIQMTQSPSSLSASVGDRVTITCRASQGIRNDLGWYQQKPGKAPKRLIYAASSLQSGVPSRFSGSGSGTEFTLTISSLQPEDCATYYCLQHNSYTWTFGQGTKVEIK

SEQ ID NO: 186 - protein, 124 aa, Homo sapiens
QVQLVESGGGVVQPGRSLRLSCVASGFTFSAYGMHWVRQAPGKGLEWVAVIWYDGSNKYYADSVKGRFIISRDNSKNTLYLQMNSLRAEDTAVYYCARSRNWNYDSYQYGLDVWGQGTTVTVSS

SEQ ID NO: 187 - protein, 11 aa, Homo sapiens
  MOD_RES (1)..(2): May or may not be present
  MOD_RES (3)..(3): Asp, Trp or absent
  MOD_RES (4)..(4): Ser, Leu or absent
  MOD_RES (5)..(5): Ile, Glu or Gln
  MOD_RES (6)..(6): Ala, Leu or Gly
  MOD_RES (7)..(7): Ala or Leu
  MOD_RES (8)..(8): Pro, Tyr or Gly
VQXXXXXXFDY

SEQ ID NO: 188 - protein, 13 aa, Homo sapiens
  MOD_RES (1)..(2): May or may not be present
  MOD_RES (3)..(3): Asp or Ala
  MOD_RES (5)..(5): Tyr or Gly
  MOD_RES (7)..(7): Ser or Tyr
  MOD_RES (8)..(8): Ser or Arg
  MOD_RES (11)..(11): May or may not be present
  MOD_RES (12)..(12): Gly or Asp
  MOD_RES (13)..(13): His or Pro
DQXYXDXXGWFXX

SEQ ID NO: 189 - protein, 9 aa, Homo sapiens
LQHNSYTWT

SEQ ID NO: 190 - protein, 10 aa, Homo sapiens
GFTFSAYGMH

SEQ ID NO: 191 - protein, 17 aa, Homo sapiens
VIWYDGSNKYYADSVKG

SEQ ID NO: 192 - protein, 15 aa, Homo sapiens
SRNWNYDSYQYGLDV

SEQ ID NO: 193 - DNA, 315 bp, Homo sapiens
tcctatgagctgactcagccaccctcagtgtccgtgtccccaggacagacagccagcatcacctgctctggagataaattgggggataaatatgtttgttggtatcagcagaagccaggccagtcccctgaactggtcatctatctagataacaagcggccctcagggatccctgagcgattctctggctccaactctgggaacacagccactctgaccatcagcgggacccaggctatggatgaggctgactattactgtcaggcgtgggacagcagcacggtattcggcggagggaccaaactgaccgtcctg

SEQ ID NO: 194 - DNA, 363 bp, Homo sapiens
caggttcagctggtgcagtctggagctgaggtgaagaagcctggggcctcagtgaaggtctcctgcaaggcttctggttacacctttaccagctatggtatcagctgggtgcgacaggcccctggacaagggcttgagaggatgggatggatcagcgcttacaatggtaacacaaactatgcacagaagttccagggcagagtcaccatgaccacagacacatcaacgaccacagcctacatggagctgaggagcctgagatctgacgacacggccgtgtattactgtgcgagagatcaagattactatgatagtagtggttggggccactggggccagggaaccctggtcaccgtctcctca

SEQ ID NO: 195 - DNA, 33 bp, Homo sapiens
tctggagataaattgggggataaatatgtttgt

SEQ ID NO: 196 - DNA, 21 bp, Homo sapiens
ctagataacaagcggccctca

SEQ ID NO: 197 - DNA, 24 bp, Homo sapiens
caggcgtgggacagcagcacggta

SEQ ID NO: 198 - DNA, 30 bp, Homo sapiens
ggttacacctttaccagctatggtatcagc

SEQ ID NO: 199 - DNA, 51 bp, Homo sapiens
tggatcagcgcttacaatggtaacacaaactatgcacagaagttccagggc

SEQ ID NO: 200 - DNA, 36 bp, Homo sapiens
gatcaagattactatgatagtagtggttggggccac

SEQ ID NO: 201 - protein, 105 aa, Homo sapiens
SYELTQPPSVSVSPGQTASITCSGDKLGDKYVCWYQQKPGQSPELVIYLDNKRPSGIPERFSGSNSGNTATLTISGTQAMDEADYYCQAWDSSTVFGGGTKLTVL

SEQ ID NO: 202 - protein, 121 aa, Homo sapiens
QVQLVQSGAEVKKPGASVKVSCKASGYTFTSYGISWVRQAPGQGLERMGWISAYNGNTNYAQKFQGRVTMTTDTSTTTAYMELRSLRSDDTAVYYCARDQDYYDSSGWGHWGQGTLVTVSS

SEQ ID NO: 203 - protein, 11 aa, Homo sapiens
SGDKLGDKYVC

SEQ ID NO: 204 - protein, 7 aa, Homo sapiens
LDNKRPS

SEQ ID NO: 205 - protein, 8 aa, Homo sapiens
QAWDSSTV

SEQ ID NO: 206 - protein, 10 aa, Homo sapiens
GYTFTSYGIS

SEQ ID NO: 207 - protein, 17 aa, Homo sapiens
WISAYNGNTNYAQKFQG

SEQ ID NO: 208 - protein, 12 aa, Homo sapiens
DQDYYDSSGWGH

SEQ ID NO: 209 - DNA, 316 bp, Homo sapiens
tcctatgagctgactcagccaccctcagtgtccgtgtccccaggacagacagcctccatcacctgctctggagataaattgggggataaatatgctttctggtatcagcagaagccaggccagtcccctgtgctggtcttctatcatgataccaagcggccctcagggatccctgagcgattctctggctccaactctgggaacacagccactctgaccatcagcgggacccaggctatggatgaggctgactatcactgtcaggcgtgggacagcagcacggtcttcggcggagggaccaagctgaccgtcctac

SEQ ID NO: 210 - DNA, 363 bp, Homo sapiens
caggttcagctggtgcaatctggagctgaggtgaagaagcctggggcctcagtgaaggtctcctgcaagacttctggttacacctttaccagctatggtatcagctgggtgcgacaggcccctggacaagggcttgagtggatgggatggatcagcccttacaatggtaacacaaactatgcacagaagttccagggcagagtcaccatgaccacagacaaatccacgagcacagcctacatggagctgaggagcctgcgatctgacgacacggccgtgtattactgtgcgagagatcaagattactatgatagtagtggttgggacccctggggccagggaaccctggtcaccgtctcctcg

SEQ ID NO: 211 - DNA, 33 bp, Homo sapiens
tctggagataaattgggggataaatatgctttc

SEQ ID NO: 212 - DNA, 21 bp, Homo sapiens
catgataccaagcggccctca

SEQ ID NO: 213 - DNA, 360 bp, Artificial Sequence
  Description of Artificial Sequence: Synthetic activin A/B chimera polynucleotide
ggtctagagtgtgatggcaaggtcaacatctgctgtaagaaacagttctttgtcagtttcaaggacatcggctggaatgactggatcattgctccctctggctatcatgccaactactgcgagggtgagtgcccgagccatatagcaggcacgtccgggtcaagcttgtccttccactcaacagtcatcaaccactaccgcatgcggggccatagcccctttgccaacctcaaatcatgctgtattcccaccaagctgagcaccatgtccatgttgtactttgatgatgagtacaacatcgtcaaaagggacgttccgaacatgatcgtggaggagtgtgggtgctcatgagcggccgct

SEQ ID NO: 214 - protein, 326 aa, Homo sapiens
ASTKGPSVFPLAPCSRSTSESTAALGCLVKDYFPEPVTVSWNSGALTSGVHTFPAVLQSSGLYSLSSVVTVPSSNFGTQTYTCNVDHKPSNTKVDKTVERKCCVECPPCPAPPVAGPSVFLFPPKPKDTLMISRTPEVTCVVVDVSHEDPEVQFNWYVDGVEVHNAKTKPREEQFNSTFRVVSVLTVVHQDWLNGKEYKCKVSNKGLPAPIEKTISKTKGQPREPQVYTLPPSREEMTKNQVSLTCLVKGFYPSDIAVEWESNGQPENNYKTTPPMLDSDGSFFLYSKLTVDKSRWQQGNVFSCSVMHEALHNHYTQKSLSLSPGK

SEQ ID NO: 215 - protein, 326 aa, Homo sapiens; identical to SEQ ID NO: 214

SEQ ID NO: 216 - DNA, 36 bp, Homo sapiens
gatcaagattactatgatagtagtggttgggacccc

SEQ ID NO: 217 - protein, 105 aa, Homo sapiens
SYELTQPPSVSVSPGQTASITCSGDKLGDKYAFWYQQKPGQSPVLVFYHDTKRPSGIPERFSGSNSGNTATLTISGTQAMDEADYHCQAWDSSTVFGGGTKLTVL

SEQ ID NO: 218 - protein, 121 aa, Homo sapiens
QVQLVQSGAEVKKPGASVKVSCKTSGYTFTSYGISWVRQAPGQGLEWMGWISPYNGNTNYAQKFQGRVTMTTDKSTSTAYMELRSLRSDDTAVYYCARDQDYYDSSGWDPWGQGTLVTVSS

SEQ ID NO: 219 - protein, 11 aa, Homo sapiens
SGDKLGDKYAF

SEQ ID NO: 220 - protein, 7 aa, Homo sapiens
HDTKRPS

SEQ ID NO: 221 - protein, 326 aa, Homo sapiens; identical to SEQ ID NO: 214

SEQ ID NO: 222 - DNA, 318 bp, Homo sapiens
ggtcagcccaaggctgccccctcggtcactctgttcccgccctcctctgaggagcttcaagccaacaaggccacactggtgtgtctcataagtgacttctacccgggagccgtgacagtggcctggaaggcagatagcagccccgtcaaggcgggagtggagaccaccacaccctccaaacaaagcaacaacaagtacgcggccagcagctatctgagcctgacgcctgagcagtggaagtcccacagaagctacagctgccaggtcacgcatgaagggagcaccgtggagaagacagtggcccctacagaatgttca

SEQ ID NO: 223 - DNA, 321 bp, Homo sapiens
cgaactgtggctgcaccatctgtcttcatcttcccgccatctgatgagcagttgaaatctggaactgcctctgttgtgtgcctgctgaataacttctatcccagagaggccaaagtacagtggaaggtggataacgccctccaatcgggtaactcccaggagagtgtcacagagcaggacagcaaggacagcacctacagcctcagcagcaccctgacgctgagcaaagcagactacgagaaacacaaagtctacgcctgcgaagtcacccatcagggcctgagctcgcccgtcacaaagagcttcaacaggggagagtgt

SEQ ID NO: 224 - protein, 12 aa, Homo sapiens
DQDYYDSSGWDP

SEQ ID NO: 225 - protein, 116 aa, Homo sapiens [sequence omitted]

SEQ ID NO: 226 - protein, 8 aa, Homo sapiens
DYKDDDDK

SEQ ID NO: 227 - DNA, 636 bp, Homo sapiens
tcctatgaggtgactcaggcaccctcagtgtccgtgtccccaggacagacagccagcatcacctgctctggagataaattgggggataaatatgcttgttggtatcagcagaagccaggccagtcccctgtgctggtcatctatcaagatagcaagcggccctcagggatccctgagcgattctctggctccaactctggaaacacagccactctgaccatcagcgggacccaggctatggatgaggctgactattactgtcaggcgtgggacagcagcactgcggtattcggcggagggaccaagctgaccgtcctaggtcagcccaaggctgccccctcggtcactctgttcccgccctcctctgaggagcttcaagccaacaaggccacactggtgtgtctcataagtgacttctacccgggagccgtgacagtggcctggaaggcagatagcagccccgtcaaggcgggagtggagaccaccacaccctccaaacaaagcaacaacaagtacgcggccagcagctatctgagcctgacgcctgagcagtggaagtcccacagaagctacagctgccaggtcacgcatgaagggagcaccgtggagaagacagtggcccctacagaatgttca

SEQ ID NO: 228 - DNA, 1344 bp, Homo sapiens
caggttcagctggtgcagtctggagctgaggtgaagaagcctggggcctcagtgaaggtctcctgcaaggcttctggttacacctttaccagttatggtctcagctgggtgcgacaggcccctggacaagggcttgagtggatgggatggatcatcccttacaatggtaacacaaactctgcacagaaactccagggcagagtcaccatgaccacagacacatccacgagcacagcctacatggagctgaggagcctgagatctgacgacacggccgtgtatttctgtgcgagagacagggactacggtgtcaattatgatgcttttgatatctggggccaagggacaatggtcaccgtctcttcagcctccaccaagggcccatcggtcttccccctggcgccctgctccaggagcacctccgagagcacagcggccctgggctgcctggtcaaggactacttccccgaaccggtgacggtgtcgtggaactcaggcgctctgaccagcggcgtgcacaccttcccagctgtcctacagtcctcaggactctactccctcagcagcgtggtgaccgtgccctccagcaacttcggcacccagacctacacctgcaacgtagatcacaagcccagcaacaccaaggtggacaagacagttgagcgcaaatgttgtgtcgagtgcccaccgtgcccagcaccacctgtggcaggaccgtcagtcttcctcttccccccaaaacccaaggacaccctcatgatctcccggacccctgaggtcacgtgcgtggtggtggacgtgagccacgaagaccccgaggtccagttcaactggtacgtggacggcgtggaggtgcataatgccaagacaaagccacgggaggagcagttcaacagcacgttccgtgtggtcagcgtcctcaccgttgtgcaccaggactggctgaacggcaaggagtacaagtgcaaggtctccaacaaaggcctcccagcccccatcgagaaaaccatctccaaaaccaaagggcagccccgagaaccacaggtgtacaccctgcccccatcccgggaggagatgaccaagaaccaggtcagcctgacctgcctggtcaaaggcttctaccccagcgacatcgccgtggagtgggagagcaatgggcagccggagaacaactacaagaccacacctcccatgctggactccgacggctccttcttcctctacagcaagctcaccgtggacaagagcaggtggcagcaggggaacgtcttctcatgctccgtgatgcatgaggctctgcacaaccactacacgcagaagagcctctccctgtctccgggtaaa

SEQ ID NO: 229 - DNA, 642 bp, Homo sapiens
gacatccagatgacccagtctccatcctccctgtctgcatctgtaggagacagagtcaccatcacttgccgggcaagtcagggcattagaaataatttaggctggtatcagcagaaaccagggaaagcccctaagcgcctgatttatgctgcatccagtttgcaaagtggggtcccatcaaggttcagcggcagtggatctgggacagaattcactctcacaatcagcagtctgcagcctgaagattttacaacttattactgtctacagcataatagttacccgtggacgttcggccaagggaccaaggtggaaatcaaacgaactgtggctgcaccatctgtcttcatcttcccgccatctgatgagcagttgaaatctggaactgcctctgttgtgtgcctgctgaataacttctatcccagagaggccaaagtacagtggaaggtggataacgccctccaatcgggtaactcccaggagagtgtcacagagcaggacagcaaggacagcacctacagcctcagcagcaccctgacgctgagcaaagcagactacgagaaacacaaagtctacgcctgcgaagtcacccatcagggcctgagctcgcccgtcacaaagagcttcaacaggggagagtgt

SEQ ID NO: 230 - DNA, 1350 bp, Homo sapiens
caggtgcagctggtggagtctgggggaggcgtggtccagcctgggaggtccctgagactctcctgtgcagcgtctggattcaccttcagtagttacggcatgcactgggtccgccaggctccaggcaaggggctggagtgggtggcagttatatggtatgatggaagtaataaataccatgcagactccgtgaagggccgattcaccatctccagagacaattccaagaacacgctgtatctgcaagtgaacagcctgagagccgaggacacggctgtgtattactgtgtgagaagtcggaactggaactacgacaactactactacggtctggacgtctggggccaagggaccacggtcaccgtctcctcagcctccaccaagggcccatcggtcttccccctggcgccctgctccaggagcacctccgagagcacagcggccctgggctgcctggtcaaggactacttccccgaaccggtgacggtgtcgtggaactcaggcgctctgaccagcggcgtgcacaccttcccagctgtcctacagtcctcaggactctactccctcagcagcgtggtgaccgtgccctccagcaacttcggcacccagacctacacctgcaacgtagatcacaagcccagcaacaccaaggtggacaagacagttgagcgcaaatgttgtgtcgagtgcccaccgtgcccagcaccacctgtggcaggaccgtcagtcttcctcttccccccaaaacccaaggacaccctcatgatctcccggacccctgaggtcacgtgcgtggtggtggacgtgagccacgaagaccccgaggtccagttcaactggtacgtggacggcgtggaggtgcataatgccaagacaaagccacgggaggagcagttcaacagcacgttccgtgtggtcagcgtcctcaccgttgtgcaccaggactggctgaacggcaaggagtacaagtgcaaggtctccaacaaaggcctcccagcccccatcgagaaaaccatctccaaaaccaaagggcagccccgagaaccacaggtgtacaccctgcccccatcccgggaggagatgaccaagaaccaggtcagcctgacctgcctggtcaaaggcttctaccccagcgacatcgccgtggagtgggagagcaatgggcagccggagaacaactacaagaccacacctcccatgctggactccgacggctccttcttcctctacagcaagctcaccgtggacaagagcaggtggcagcaggggaacgtcttctcatgctccgtgatgcatgaggctctgcacaaccactacacgcagaagagcctctccctgtctccgggtaaa

SEQ ID NO: 231 - DNA, 642 bp, Homo sapiens
gacatccagatgacccagtctccatcctccctgtctgcatctgtaggagacagagtcaccatcacttgccgggcaagtcagggcattagaaatgatttaggctggtatcagcagaaaccagggaaagcccctaagcgcctgatctatgctgcatccagtttgcaaagtggggtcccatcaaggttcagcggcagtggatctgggacagaattcactctcacaatcagcagcctgcagcctgaagattttgcaacttattactgtcgacagcaaaatacttacccgctcactttcggcggagggaccaaggtggagatcaaacgaactgtggctgcaccatctgtcttcatcttcccgccatctgatgagcagttgaaatctggaactgcctctgttgtgtgcctgctgaataacttctatcccagagaggccaaagtacagtggaaggtggataacgccctccaatcgggtaactcccaggagagtgtcacagagcaggacagcaaggacagcacctacagcctcagcagcaccctgacgctgagcaaagcagactacgagaaacacaaagtctacgcctgcgaagtcacccatcagggcctgagctcgcccgtcacaaagagcttcaacaggggagagtgt

SEQ ID NO: 232 - DNA, 1347 bp, Homo sapiens
gaggtgcagttggtggagtctgggggaggcttggtccagcctggggggtccctgagactctcctgtgcagcctctggattcacctttagtagttattggatgagctgggtccgccaggctccagggaaggggctggagtgcgtggccaacataaagcaagatggaagtgaggaatactatgtggactctgtgaagggccgattcaccatctccagagacaacgccaagaattcactgtatctgcaaatgaacagcctgagagccgaggacacggctgtgtattactgtgcgagaggtagcagcagctggtactactacaactacggtatggacgtctggggccaagggaccacggtcaccgtctcctcagcctccaccaagggcccatcggtcttccccctggcgccctgctccaggagcacctccgagagcacagcggccctgggctgcctggtcaaggactacttccccgaaccggtgacggtgtcgtggaactcaggcgctctgaccagcggcgtgcacaccttcccagctgtcctacagtcctcaggactctactccctcagcagcgtggtgaccgtgccctccagcaacttcggcacccagacctacacctgcaacgtagatcacaagcccagcaacaccaaggtggacaagacagttgagcgcaaatgttgtgtcgagtgcccaccgtgcccagcaccacctgtggcaggaccgtcagtcttcctcttccccccaaaacccaaggacaccctcatgatctcccggacccctgaggtcacgtgcgtggtggtggacgtgagccacgaagaccccgaggtccagttcaactggtacgtggacggcgtggaggtgcataatgccaagacaaagccacgggaggagcagttcaacagcacgttccgtgtggtcagcgtcctcaccgttgtgcaccaggactggctgaacggcaaggagtacaagtgcaaggtctccaacaaaggcctcccagcccccatcgagaaaaccatctccaaaaccaaagggcagccccgagaaccacaggtgtacaccctgcccccatcccgggaggagatgaccaagaaccaggtcagcctgacctgcctggtcaaaggcttctaccccagcgacatcgccgtggagtgggagagcaatgggcagccggagaacaactacaagaccacacctcccatgctggactccgacggctccttcttcctctacagcaagctcaccgtggacaagagcaggtggcagcaggggaacgtcttctcatgctccgtgatgcatgaggctctgcacaaccactacacgcagaagagcctctccctgtctccgggtaaa

SEQ ID NO: 233 - protein, 212 aa, Homo sapiens
SYEVTQAPSVSVSPGQTASITCSGDKLGDKYACWYQQKPGQSPVLVIYQDSKRPSGIPERFSGSNSGNTATLTISGTQAMDEADYYCQAWDSSTAVFGGGTKLTVLGQPKAAPSVTLFPPSSEELQANKATLVCLISDFYPGAVTVAWKADSSPVKAGVETTTPSKQSNNKYAASSYLSLTPEQWKSHRSYSCQVTHEGSTVEKTVAPTECS

SEQ ID NO: 234 - protein, 448 aa, Homo sapiens
QVQLVQSGAEVKKPGASVKVSCKASGYTFTSYGLSWVRQAPGQGLEWMGWIIPYNGNTNSAQKLQGRVTMTTDTSTSTAYMELRSLRSDDTAVYFCARDRDYGVNYDAFDIWGQGTMVTVSSASTKGPSVFPLAPCSRSTSESTAALGCLVKDYFPEPVTVSWNSGALTSGVHTFPAVLQSSGLYSLSSVVTVPSSNFGTQTYTCNVDHKPSNTKVDKTVERKCCVECPPCPAPPVAGPSVFLFPPKPKDTLMISRTPEVTCVVVDVSHEDPEVQFNWYVDGVEVHNAKTKPREEQFNSTFRVVSVLTVVHQDWLNGKEYKCKVSNKGLPAPIEKTISKTKGQPREPQVYTLPPSREEMTKNQVSLTCLVKGFYPSDIAVEWESNGQPENNYKTTPPMLDSDGSFFLYSKLTVDKSRWQQGNVFSCSVMHEALHNHYTQKSLSLSPGK

SEQ ID NO: 235 - protein, 214 aa, Homo sapiens
DIQMTQSPSSLSASVGDRVTITCRASQGIRNNLGWYQQKPGKAPKRLIYAASSLQSGVPSRFSGSGSGTEFTLTISSLQPEDFTTYYCLQHNSYPWTFGQGTKVEIKRTVAAPSVFIFPPSDEQLKSGTASVVCLLNNFYPREAKVQWKVDNALQSGNSQESVTEQDSKDSTYSLSSTLTLSKADYEKHKVYACEVTHQGLSSPVTKSFNRGEC

SEQ ID NO: 236 - protein, 450 aa, Homo sapiens
QVQLVESGGGVVQPGRSLRLSCAASGFTFSSYGMHWVRQAPGKGLEWVAVIWYDGSNKYHADSVKGRFTISRDNSKNTLYLQVNSLRAEDTAVYYCVRSRNWNYDNYYYGLDVWGQGTTVTVSSASTKGPSVFPLAPCSRSTSESTAALGCLVKDYFPEPVTVSWNSGALTSGVHTFPAVLQSSGLYSLSSVVTVPSSNFGTQTYTCNVDHKPSNTKVDKTVERKCCVECPPCPAPPVAGPSVFLFPPKPKDTLMISRTPEVTCVVVDVSHEDPEVQFNWYVDGVEVHNAKTKPREEQFNSTFRVVSVLTVVHQDWLNGKEYKCKVSNKGLPAPIEKTISKTKGQPREPQVYTLPPSREEMTKNQVSLTCLVKGFYPSDIAVEWESNGQPENNYKTTPPMLDSDGSFFLYSKLTVDKSRWQQGNVFSCSVMHEALHNHYTQKSLSLSPGK

SEQ ID NO: 237 - protein, 214 aa, Homo sapiens
DIQMTQSPSSLSASVGDRVTITCRASQGIRNDLGWYQQKPGKAPKRLIYAASSLQSGVPSRFSGSGSGTEFTLTISSLQPEDFATYYCRQQNTYPLTFGGGTKVEIKRTVAAPSVFIFPPSDEQLKSGTASVVCLLNNFYPREAKVQWKVDNALQSGNSQESVTEQDSKDSTYSLSSTLTLSKADYEKHKVYACEVTHQGLSSPVTKSFNRGEC

SEQ ID NO: 238 - protein, 449 aa, Homo sapiens
EVQLVESGGGLVQPGGSLRLSCAASGFTFSSYWMSWVRQAPGKGLECVANIKQDGSEEYYVDSVKGRFTISRDNAKNSLYLQMNSLRAEDTAVYYCARGSSSWYYYNYGMDVWGQGTTVTVSSASTKGPSVFPLAPCSRSTSESTAALGCLVKDYFPEPVTVSWNSGALTSGVHTFPAVLQSSGLYSLSSVVTVPSSNFGTQTYTCNVDHKPSNTKVDKTVERKCCVECPPCPAPPVAGPSVFLFPPKPKDTLMISRTPEVTCVVVDVSHEDPEVQFNWYVDGVEVHNAKTKPREEQFNSTFRVVSVLTVVHQDWLNGKEYKCKVSNKGLPAPIEKTISKTKGQPREPQVYTLPPSREEMTKNQVSLTCLVKGFYPSDIAVEWESNGQPENNYKTTPPMLDSDGSFFLYSKLTVDKSRWQQGNVFSCSVMHEALHNHYTQKSLSLSPGK

SEQ ID NO: 239 - DNA, 321 bp, Homo sapiens; identical to SEQ ID NO: 223

SEQ ID NO: 240 - DNA, 978 bp, Homo sapiens
gcctccaccaagggcccatcggtcttccccctggcgccctgctccaggagcacctccgagagcacagcggccctgggctgcctggtcaaggactacttccccgaaccggtgacggtgtcgtggaactcaggcgctctgaccagcggcgtgcacaccttcccagctgtcctacagtcctcaggactctactccctcagcagcgtggtgaccgtgccctccagcaacttcggcacccagacctacacctgcaacgtagatcacaagcccagcaacaccaaggtggacaagacagttgagcgcaaatgttgtgtcgagtgcccaccgtgcccagcaccacctgtggcaggaccgtcagtcttcctcttccccccaaaacccaaggacaccctcatgatctcccggacccctgaggtcacgtgcgtggtggtggacgtgagccacgaagaccccgaggtccagttcaactggtacgtggacggcgtggaggtgcataatgccaagacaaagccacgggaggagcagttcaacagcacgttccgtgtggtcagcgtcctcaccgttgtgcaccaggactggctgaacggcaaggagtacaagtgcaaggtctccaacaaaggcctcccagcccccatcgagaaaaccatctccaaaaccaaagggcagccccgagaaccacaggtgtacaccctgcccccatcccgggaggagatgaccaagaaccaggtcagcctgacctgcctggtcaaaggcttctaccccagcgacatcgccgtggagtgggagagcaatgggcagccggagaacaactacaagaccacacctcccatgctggactccgacggctccttcttcctctacagcaagctcaccgtggacaagagcaggtggcagcaggggaacgtcttctcatgctccgtgatgcatgaggctctgcacaaccactacacgcagaagagcctctccctgtctccgggtaaa

SEQ ID NO: 241 - DNA, 978 bp, Homo sapiens; identical to SEQ ID NO: 240

SEQ ID NO: 242 - DNA, 824 bp, Homo sapiens
gcctccaccaagggcccatcggtcttccccctggcgccctgctccaggagcacctccgagagcacagcggccctgggctgcctggtcaaggactacttccccgaaccggtgacggtgtcgtggaactcaggcgctctgaccagcggcgtgcacaccttcccagctgtcctacagtcctcaggactctactccctcagcagcgtggtgaccgtgccctccagcaacttcggcacccagacctacacctgcaacgtagatcacaagcccagcaacaccaaggtggacaagacagttgagcgcaaatgttgtgtcgagtgcccaccgtgcccagcaccacctgtggcaggaccgtcagtcttcctcttccccccaaaacccaaggacaccctcatgatctcccggacccctgaggtcacgtgcgtggtggtggacgtgagccacgaagaccccgaggtccagttcaactggtacgtggacggcgtggaggtgcataatgccaagacaaagccacgggaggagcagttcaacagcacgttccgtgtggtcagcgtcctcaccgttgtgcaccaggactggctgaacggcaaggagtacaagtgcaaggtctccaacaaaggcctcccagcccccatcgagaaaaccatctccaaaaccaaagggcagccccgagaaccacaggtgtacaccctgcccccatcccgggaggagatgaccaagaaccaggtcagcctgacctgcctggtcaaaggcttctaccccagcgacatcgccgtggagtgggagagcaatgggcagccggagaacaactacaagaccacacctcc

SEQ ID NO: 243 - protein, 116 aa, Artificial Sequence
  Description of Artificial Sequence: Synthetic activin A/B chimera polypeptide
GLECDGKVNICCRQQFFIDFRLIGWNDWIIAPTGYYGNYCEGECPSHIAGTSGSSLSFHSTVINHYRMRGHSPFANLKSCCVPTKLRPMSMLYYDDGQNIIKKDIQNMIVEECGCS

SEQ ID NO: 244 - protein, 116 aa, Artificial Sequence
  Description of Artificial Sequence: Synthetic activin A/B chimera polypeptide
GLECDGKVNICCKKQFFVSFKDIGWNDWIIAPSGYHANYCEGECPSHIAGTSGSSLSFHSTVINHYRMRGHSPFANLKSCCIPTKLSTMSMLYFDDEYNIVKRDVPNMIVEECGCS

SEQ ID NO: 245 - DNA, 31 bp, Artificial Sequence
  Description of Artificial Sequence: Synthetic oligonucleotide
ctcgaggtcgactagaccaccatgcccttgc

SEQ ID NO: 246 - DNA, 28 bp, Artificial Sequence
  Description of Artificial Sequence: Synthetic oligonucleotide
ccatcacactctagaccccgccgacgcc

SEQ ID NO: 247 - DNA, 360 bp, Artificial Sequence
  Description of Artificial Sequence: Synthetic activin A/B chimera polynucleotide
ggtctagagtgtgatggcaaggtcaacatctgctgtaggcaacagttctttatcgatttcaggctcatcggctggaatgactggatcattgctcccactggctattatggcaactactgcgagggtgagtgcccgagccatatagcaggcacgtccgggtcaagcttgtccttccactcaacagtcatcaaccactaccgcatgcggggccatagcccctttgccaacctcaaatcatgctgtgtgcccaccaagctgagacccatgtccatgttgtactatgatgatggtcaaaacatcatcaaaaaggacattcagaacatgatcgtggaggagtgtgggtgctcatgagcggccgct

SEQ ID NO: 248 - protein, 9 aa, Artificial Sequence
  Description of Artificial Sequence: Synthetic anti activin A antibody peptide
  MOD_RES (5)..(5): Arg or Ser
  MOD_RES (8)..(8): Val or Ala
  MOD_RES (9)..(9): May or may not be present
QAWDXSTXV

SEQ ID NO: 249 - protein, 16 aa, Artificial Sequence
  Description of Artificial Sequence: Synthetic anti activin A antibody peptide
  MOD_RES (1)..(1): May or may not be present
  MOD_RES (2)..(2): Ser, Glu or absent
  MOD_RES (3)..(3): Arg, Ser or absent
  MOD_RES (4)..(4): Asp, Asn, Ser or Gln
  MOD_RES (5)..(5): Ser, Arg or Trp
  MOD_RES (6)..(6): Gly, Asp, Asn, Tyr or Leu
  MOD_RES (8)..(8): Ser, Gly, Asp or absent
  MOD_RES (9)..(9): Ser, Val, Asn or Tyr
  MOD_RES (10)..(10): Ser, Asn, Tyr or His
  MOD_RES (11)..(11): Trp, Tyr or Gln
  MOD_RES (12)..(12): His, Asp, Tyr or absent
  MOD_RES (13)..(13): Phe, Ala or Gly
  MOD_RES (14)..(14): Asp, Phe, Leu or Met
  MOD_RES (15)..(15): Tyr or Asp
  MOD_RES (16)..(16): Ile, Val or absent
GXXXXXYXXXXXXXXX

SEQ ID NO: 250 - protein, 11 aa, Artificial Sequence
  Description of Artificial Sequence: Synthetic anti activin A antibody peptide
  MOD_RES (3)..(3): Ser or Gly
  MOD_RES (7)..(7): Ser or Arg
  MOD_RES (9)..(9): Asp or Asn
  MOD_RES (11)..(11): Val or Gly
RAXQGIXNXLX

SEQ ID NO: 251 - protein, 12 aa, Artificial Sequence
  Description of Artificial Sequence: Synthetic anti activin A antibody peptide
RASQSISNYLNT

SEQ ID NO: 252 - protein, 12 aa, Artificial Sequence
  Description of Artificial Sequence: Synthetic anti activin A antibody peptide
  MOD_RES (4)..(4): Ile or Phe
  MOD_RES (5)..(5): Asn or Ser
  MOD_RES (6)..(6): Ser or Ala
  MOD_RES (7)..(8): May or may not be present
  MOD_RES (9)..(9): Phe or Tyr
GGSXXXGGXYWS

SEQ ID NO: 253 - protein, 16 aa, Artificial Sequence
  Description of Artificial Sequence: Synthetic anti activin A antibody peptide
RSSQSLLHSTGYNYLD

SEQ ID NO: 254 - protein, 7 aa, Artificial Sequence
  Description of Artificial Sequence: Synthetic anti activin A antibody peptide
LGSFRAS

SEQ ID NO: 255 - protein, 9 aa, Artificial Sequence
  Description of Artificial Sequence: Synthetic anti activin A antibody peptide
MQALQTPCS

SEQ ID NO: 256 - protein, 10 aa, Artificial Sequence
  Description of Artificial Sequence: Synthetic anti activin A antibody peptide
GYTFTGYYIH

SEQ ID NO: 257 - protein, 10 aa, Artificial Sequence
  Description of Artificial Sequence: Synthetic anti activin A antibody peptide
  MOD_RES (2)..(2): Tyr or Phe
  MOD_RES (3)..(3): Thr or Ser
  MOD_RES (5)..(5): Thr,Ser or Ile
  MOD_RES (6)..(6): Gly or Ser
  MOD_RES (8)..(8): Tyr, Gly or Trp
  MOD_RES (9)..(9): Ile or Met
  MOD_RES (10)..(10): His or Gly
GXXFXXYXXX

SEQ ID NO: 258 - protein, 17 aa, Artificial Sequence
  Description of Artificial Sequence: Synthetic anti activin A antibody peptide
WINPNSGGTNYAQKFQG

SEQ ID NO: 259 - protein, 17 aa, Artificial Sequence
  Description of Artificial Sequence: Synthetic anti activin A antibody peptide
WISPYNGNTNYAQKFQG

SEQ ID NO: 260 - protein, 12 aa, Artificial Sequence
  Description of Artificial Sequence: Synthetic anti activin A antibody peptide
DSGYSSSWHFDY

SEQ ID NO: 261 - protein, 13 aa, Artificial Sequence
  Description of Artificial Sequence: Synthetic anti activin A antibody peptide
GSSSWYYYNGMDV

SEQ ID NO: 262 - protein, 30 aa, Artificial Sequence
  Description of Artificial Sequence: Synthetic polypeptide corresponding to amino acid residues 1-30 of activin A
GLECDGKVNICCKKQFFVSFKDIGWNDWII

SEQ ID NO: 263 - protein, 30 aa, Artificial Sequence
  Description of Artificial Sequence: Synthetic polypeptide corresponding to amino acid residues 31-60 of activin A
APSGYHANYCEGECPSHIAGTSGSSLSFHS

SEQ ID NO: 264 - protein, 30 aa, Artificial Sequence
  Description of Artificial Sequence: Synthetic polypeptide corresponding to amino acid residues 61-90 of activin A
TVINHYRMRGHSPFANLKSCCVPTKLRPMS

SEQ ID NO: 265 - protein, 26 aa, Artificial Sequence
  Description of Artificial Sequence: Synthetic peptide corresponding to amino acid residues 91-116 of activin A
MLYYDDGQNIIKKDIQNMIVEECGCS

SEQ ID NO: 266 - protein, 116 aa, Artificial Sequence; identical to SEQ ID NO: 243
  Description of Artificial Sequence: Synthetic activin A 13/39B polypeptide

SEQ ID NO: 267 - DNA, 318 bp, Homo sapiens
tcctatgaggtgactcaggcaccctcagtgtccgtgtccccaggacagacagccagcatcacctgctctggagataaattgggggataaatatgcttgttggtatcagcagaagccaggccagtcccctgtgctggtcatctatcaagatagcaagcggccctcagggatccctgagcgattctctggctccaactctggaaacacagccactctgaccatcagcgggacccaggctatggatgaggctgactattactgtcaggcgtgggacagcagcactgcggtattcggcggagggaccaagctgaccgtccta

SEQ ID NO: 268 - DNA, 366 bp, Homo sapiens
caggttcagctggtgcagtctggagctgaggtgaagaagcctggggcctcagtgaaggtctcctgcaaggcttctggttacacctttaccagttatggtctcagctgggtgcgacaggcccctggacaagggcttgagtggatgggatggatcatcccttacaatggtaacacaaactctgcacagaaactccagggcagagtcaccatgaccacagacacatccacgagcacagcctacatggagctgaggagcctgagatctgacgacacggccgtgtatttctgtgcgagagacagggactacggtgtcaattatgatgcttttgatatctggggccaagggacaatggtcaccgtctcttca

SEQ ID NO: 269 - DNA, 373 bp, Homo sapiens
caggtgcagctggtggagtctgggggaggcgtggtccagcctgggaggtccctgagactctcctgtgcagcgtctggattcaccttcagtagttacggcatgcactgggtccgccaggctccaggcaaggggctggagtgggtggcagttatatggtatgatggaagtaataaataccatgcagactccgtgaagggccgattcaccatctccagagacaattccaagaacacgctgtatctgcaagtgaacagcctgagagccgaggacacggctgtgtattactgtgtgagaagtcggaactggaactacgacaactactactacggtctggacgtctggggccaagggaccacggtcaccgtctcctcag

SEQ ID NO: 270 - DNA, 321 bp, Homo sapiens
gacatccagatgacccagtctccatcctccctgtctgcatctgtaggagacagagtcaccatcacttgccgggcaagtcagggcattagaaataatttaggctggtatcagcagaaaccagggaaagcccctaagcgcctgatttatgctgcatccagtttgcaaagtggggtcccatcaaggttcagcggcagtggatctgggacagaattcactctcacaatcagcagtctgcagcctgaagattttacaacttattactgtctacagcataatagttacccgtggacgttcggccaagggaccaaggtggaaatcaaa

SEQ ID NO: 271 - DNA, 369 bp, Homo sapiens
gaggtgcagttggtggagtctgggggaggcttggtccagcctggggggtccctgagactctcctgtgcagcctctggattcacctttagtagttattggatgagctgggtccgccaggctccagggaaggggctggagtgcgtggccaacataaagcaagatggaagtgaggaatactatgtggactctgtgaagggccgattcaccatctccagagacaacgccaagaattcactgtatctgcaaatgaacagcctgagagccgaggacacggctgtgtattactgtgcgagaggtagcagcagctggtactactacaactacggtatggacgtctggggccaagggaccacggtcaccgtctcctca

SEQ ID NO: 272 - DNA, 321 bp, Homo sapiens
gacatccagatgacccagtctccatcctccctgtctgcatctgtaggagacagagtcaccatcacttgccgggcaagtcagggcattagaaatgatttaggctggtatcagcagaaaccagggaaagcccctaagcgcctgatctatgctgcatccagtttgcaaagtggggtcccatcaaggttcagcggcagtggatctgggacagaattcactctcacaatcagcagcctgcagcctgaagattttgcaacttattactgtcgacagcaaaatacttacccgctcactttcggcggagggaccaaggtggagatcaaa

SEQ ID NO: 273 - DNA, 363 bp, Homo sapiens
caggtgcagctggtgcagtctggggctgaggtgaagaagcctggggcctcagtgaaggtctcctgcaaggcttctggatacaccttcaccggctactatatccactgggtgcgacaggcccctggacaagggcttgagtggatgggatggatcaaccctaacagtggtggcacaaactatgcacagaagtttcagggcagggtcaccatgaccagggacacgtccatcagcacagcctacatggagctgagcaggctgagatctgacgacacggccgtgtatttctgtgcgagagattcggggtatagcagcagctggcactttgactactggggccagggaaccctggtcaccgtctcctca

SEQ ID NO: 274 - DNA, 336 bp, Homo sapiens
gatattgtgatgactcagtctccactctccctgcccgtcacccctggagagccggcctccatctcctgcaggtctagtcagagcctcctgcatagtactggatacaactatttggattggtacctgcagaagccagggcagtctccacagctcctgatctatttgggttcttttcgggcctccggggtccctgacaggttcagtggcagtgggtcaggcacagattttacactgaaaatcagcagagtggaggctgaggatgttggggtttattactgcatgcaagctctccaaactccgtgcagttttggccaggggaccaagctggagatcaag

SEQ ID NO: 275 - protein, 106 aa, Homo sapiens
SYEVTQAPSVSVSPGQTASITCSGDKLGDKYACWYQQKPGQSPVLVIYQDSKRPSGIPERFSGSNSGNTATLTISGTQAMDEADYYCQAWDSSTAVFGGGTKLTVL

SEQ ID NO: 276 - protein, 107 aa, Homo sapiens; identical to SEQ ID NO: 137

SEQ ID NO: 277 - protein, 107 aa, Homo sapiens
DIQMTQSPSSLSASVGDRVTITCRASQGIRNDLGWYQQKPGKAPKRLIYAASSLQSGVPSRFSGSGSGTEFTLTISSLQPEDFATYYCRQQNTYPLTFGGGTKVEIK

SEQ ID NO: 278 - protein, 122 aa, Homo sapiens
QVQLVQSGAEVKKPGASVKVSCKASGYTFTSYGLSWVRQAPGQGLEWMGWIIPYNGNTNSAQKLQGRVTMTTDTSTSTAYMELRSLRSDDTAVYFCARDRDYGVNYDAFDIWGQGTMVTVSS

SEQ ID NO: 279 - protein, 124 aa, Homo sapiens; identical to SEQ ID NO: 138

SEQ ID NO: 280 - protein, 123 aa, Homo sapiens
EVQLVESGGGLVQPGGSLRLSCAASGFTFSSYWMSWVRQAPGKGLECVANIKQDGSEEYYVDSVKGRFTISRDNAKNSLYLQMNSLRAEDTAVYYCARGSSSWYYYNYGMDVWGQGTTVTVSS

SEQ ID NO: 281 - protein, 11 aa, Homo sapiens
RASQGIRNNLG

SEQ ID NO: 282 - protein, 11 aa, Homo sapiens
RASQGIRNDLG

SEQ ID NO: 283 - protein, 7 aa, Homo sapiens
AASSLQS

SEQ ID NO: 284 - protein, 9 aa, Homo sapiens
RQQNTYPLT

SEQ ID NO: 285 - protein, 10 aa, Homo sapiens
GFTFSSYGMH

SEQ ID NO: 286 - protein, 10 aa, Homo sapiens
GFTFSSYWMS

SEQ ID NO: 287 - protein, 17 aa, Homo sapiens
NIKQDGSEEYYVDSVKG

SEQ ID NO: 288 - protein, 14 aa, Homo sapiens
GSSSWYYYNYGMDV

SEQ ID NO: 289 - protein, 5 aa, Artificial Sequence
  Description of Artificial Sequence: Synthetic peptide
GGGGG

SEQ ID NO: 290 - protein, 8 aa, Artificial Sequence
  Description of Artificial Sequence: Synthetic peptide
GGGGGGGG

SEQ ID NO: 291 - DNA, 21 bp, Artificial Sequence
  Description of Artificial Sequence: Synthetic primer
gaaaaggagcagtcgcacaga

SEQ ID NO: 292 - DNA, 19 bp, Artificial Sequence
  Description of Artificial Sequence: Synthetic primer
cttctggtgggagtagcgg

SEQ ID NO: 293 - DNA, 20 bp, Artificial Sequence
  Description of Artificial Sequence: Synthetic probe
atgctgcaggcccggcagtc

SEQ ID NO: 294 - DNA, 21 bp, Artificial Sequence
  Description of Artificial Sequence: Synthetic primer
cccttgctttggctgagagga

SEQ ID NO: 295 - DNA, 20 bp, Artificial Sequence
  Description of Artificial Sequence: Synthetic primer
tcacaggtcgtcgtaggtcg

SEQ ID NO: 296 - DNA, 17 bp, Artificial Sequence
  Description of Artificial Sequence: Synthetic primer
tgtgccggggagaagag

SEQ ID NO: 297 - DNA, 21 bp, Artificial Sequence
  Description of Artificial Sequence: Synthetic primer
tacagtagtgggttgaggttc

SEQ ID NO: 298 - DNA, 33 bp, Homo sapiens
tctggagataaattgggggataaatatgcttgt

SEQ ID NO: 299 - DNA, 21 bp, Homo sapiens
caagatagcaagcggccctca

SEQ ID NO: 300 - DNA, 27 bp, Homo sapiens
caggcgtgggacagcagcactgcggta

SEQ ID NO: 301 - DNA, 30 bp, Homo sapiens
ggttacacctttaccagttatggtctcagc

SEQ ID NO: 302 - DNA, 51 bp, Homo sapiens
tggatcatcccttacaatggtaacacaaactctgcacagaaactccagggc

SEQ ID NO: 303 - DNA, 39 bp, Homo sapiens
gacagggactacggtgtcaattatgatgcttttgatatc

SEQ ID NO: 304 - DNA, 33 bp, Homo sapiens
cgggcaagtcagggcattagaaataatttaggc

SEQ ID NO: 305 - DNA, 21 bp, Homo sapiens
gctgcatccagtttgcaaagt

SEQ ID NO: 306 - DNA, 30 bp, Homo sapiens
ggattcaccttcagtagttacggcatgcac

SEQ ID NO: 307 - DNA, 33 bp, Homo sapiens
cgggcaagtcagggcattagaaatgatttaggc

SEQ ID NO: 308 - DNA, 21 bp, Homo sapiens
gctgcatccagtttgcaaagt

SEQ ID NO: 309 - DNA, 27 bp, Homo sapiens
cgacagcaaaatacttacccgctcact

SEQ ID NO: 310 - DNA, 30 bp, Homo sapiens
ggattcacctttagtagttattggatgagc

SEQ ID NO: 311 - DNA, 51 bp, Homo sapiens
aacataaagcaagatggaagtgaggaatactatgtggactctgtgaagggc

SEQ ID NO: 312 - DNA, 42 bp, Homo sapiens
ggtagcagcagctggtactactacaactacggtatggacgtc